European Patent Specification EP 3 624 824 B1, published July 10, 2024. Title: TREATMENT OF CYSTIC FIBROSIS BY DELIVERY OF CODON-OPTIMIZED mRNA ENCODING CFTR. Applicant: Translate Bio Inc. Application Not yet determined. The sequence listing filed with the application follows.

SEQUENCE LISTING (27 sequences)

SEQ ID NO: 1 - RNA, 4443 nt, Artificial Sequence
  Chemically Synthesized Oligonucleotide
augcaacgcucuccucuugaaaaggccucggugguguccaagcucuucuucucguggacuagacccauccugagaaagggguacagacagcgcuuggagcuguccgauaucuaucaaaucccuuccguggacuccgcggacaaccuguccgagaagcucgagagagaaugggacagagaacucgccucaaagaagaacccgaagcugauuaaugcgcuuaggcggugcuuuuucuggcgguucauguucuacggcaucuuccucuaccugggagaggucaccaaggccgugcagccccuguugcugggacggauuauugccuccuacgaccccgacaacaaggaagaaagaagcaucgcuaucuacuugggcaucggucugugccugcuuuucaucguccggacccucuuguugcauccugcuauuuucggccugcaucacauuggcaugcagaugagaauugccauguuuucccugaucuacaagaaaacucugaagcucucgagccgcgugcuugacaagauuuccaucggccagcucgugucccugcucuccaacaaucugaacaaguucgacgagggccucgcccuggcccacuucguguggaucgccccucugcaaguggcgcuucugaugggccugaucugggagcugcugcaagccucggcauucugugggcuuggauuccugaucgugcuggcacuguuccaggccggacuggggcggaugaugaugaaguacagggaccagagagccggaaagauuuccgaacggcuggugaucacuucggaaaugaucgaaaacauccagucagugaaggccuacugcugggaagaggccauggaaaagaugauugaaaaccuccggcaaaccgagcugaagcugacccgcaaggccgcuuacgugcgcuauuucaacucguccgcuuucuucuucuccggguucuucgugguguuucucuccgugcuccccuacgcccugauuaagggaaucauccucaggaagaucuucaccaccauuuccuucuguaucgugcuccgcauggccgugacccggcaguucccaugggccgugcagacuugguacgacucccugggagccauuaacaagauccaggacuuccuucaaaagcaggaguacaagacccucgaguacaaccugacuacuaccgaggucgugauggaaaacgucaccgccuuuugggaggagggauuuggcgaacuguucgagaaggccaagcagaacaacaacaaccgcaagaccucgaacggugacgacucccucuucuuuucaaacuucagccugcucgggacgcccgugcugaaggacauuaacuucaagaucgaaagaggacagcuccuggcgguggccggaucgaccggagccggaaagacuucccugcugauggugaucaugggagagcuugaaccuagcgagggaaagaucaagcacuccggccgcaucagcuucuguagccaguuuuccuggaucaugcccggaaccauuaaggaaaacaucaucuucggcguguccuacgaugaauaccgcuaccgguccgugaucaaagccugccagcuggaagaggauauuucaaaguucgcggagaaagauaacaucgugcugggcgaaggggguauuaccuugucggggggccagcgggcuagaaucucgcuggccagagccguguauaaggacgccgaccuguaucuccuggacucccccuucggauaccuggacguccugaccgaaaaggagaucuucgaaucgugcgugugcaagcugauggcuaacaagacucgcauccucgugaccuccaaaauggagcaccugaagaaggcagacaagauucugauucugcaugagggguccuccuacuuuuacggcaccuucucggaguugcagaacuugcagcccgacuucucaucgaagcugauggguugcgacagcuucgaccaguucuccgccgaaagaaggaacucgauccugacggaaaccuugcaccgcuucucuuuggaaggcgacgccccugugucauggaccgagacuaagaagcagagcuucaagcagaccggggaauucggcgaaaagaggaagaacagcaucuugaaccccauuaacuccauccgcaaguucucaaucgugcaaaagacgccacugcagaugaacggcauugaggaggacuccgacgaaccccuugagaggcgccugucccuggugccggacagcgagcagggagaagccauccugccucggauuuccgugaucuccacugguccgacgcuccaagcccggcggcggcaguccgugcugaaccugaugacccacagcgugaaccagggccaaaacauucaccgcaagacuaccgcauccacccggaaagugucccuggcaccucaagcgaaucuuaccgagcucgacaucuacucccggagacugucgcaggaaaccgggcucgaaauuuccgaagaaaucaacgaggaggaucugaaagagugcuucuucgacgauauggagucgauacccgccgugacgacuuggaacacuuaucugcgguacaucacugugcacaagucauugaucuucgugcugauuuggugccuggugauuuuccuggccgaggucgcggccucacugguggugcucuggcuguugggaaacacgccucugcaagacaagggaaacuccacgcacucgagaaacaacagcuaugccgugauuaucacuuccaccuccucuuauuacguguucuacaucuacgucggaguggcggauacccugcucgcgauggguuucuucagaggacugccgcugguccacaccuugaucaccgucagcaagauucuucaccacaagauguugcauagcgugcugcaggcccccauguccacccucaacacucugaaggccggaggcauucugaacagauucuccaaggacaucgcuauccuggacgaucuccugccgcuuaccaucuuugacuucauccagcugcugcugaucgugauuggagcaaucgcagugguggcggugcugcagccuuacauuuucguggccacugugccggucauuguggcguucaucaugcugcgggccuacuuccuccaaaccagccagcagcugaagcaacuggaauccgagggacgaucccccaucuucacucaccuugugacgucguugaagggacuguggacccuccgggcuuucggacggcagcccuacuucgaaacccucuuccacaaggcccugaaccuccacaccgccaauugguuccuguaccuguccacccugcggugguuccagaugcgcaucgagaugauuuucgucaucuucuucaucgcggucacauucaucagcauccugacuaccggagagggagagggacgggucggaauaauccugacccucgccaugaacauuaugagcacccugcagugggcagugaacagcucgaucgacguggacagccugaugcgaagcgucagccgcguguucaaguucaucgacaugccuacugagggaaaacccacuaaguccacuaagcccuacaaaaauggccagcugagcaaggucaugaucaucgaaaacucccacgugaagaaggacgauauuuggcccuccggaggucaaaugaccgugaaggaccugaccgcaaaguacaccgagggaggaaacgccauucucgaaaacaucagcuucuccauuucgccgggacagcgggucggccuucucgggcggaccgguuccgggaagucaacucugcugucggcuuuccuccggcugcugaauaccgagggggaaauccaaauugacggcgugucuugggauuccauuacucugcagcaguggcggaaggccuucggcgugaucccccagaagguguucaucuucucggguaccuuccggaagaaccuggauccuuacgagcaguggagcgaccaagaaaucuggaaggucgccgacgaggucggccugcgcuccgugauugaacaauuuccuggaaagcuggacuucgugcucgucgacgggggauguguccugucgcacggacauaagcagcucaugugccucgcacgguccgugcucuccaaggccaagauucugcugcuggacgaaccuucggcccaccuggauccggucaccuaccagaucaucaggaggacccugaagcaggccuuugccgauugcaccgugauucucugcgagcaccgcaucgaggccaugcuggagugccagcaguuccuggucaucgaggagaacaagguccgccaauacgacuccauucaaaagcuccucaacgagcggucgcuguucagacaagcuauuucaccguccgauagagugaagcucuucccgcaucggaacagcucaaagugcaaaucgaagccgcagaucgcagccuugaaggaagagacugaggaagaggugcaggacacccggcuuuaa

SEQ ID NO: 2 - protein, 1480 aa, Homo sapiens
MQRSPLEKASVVSKLFFSWTRPILRKGYRQRLELSDIYQIPSVDSADNLSEKLEREWDRELASKKNPKLINALRRCFFWRFMFYGIFLYLGEVTKAVQPLLLGRIIASYDPDNKEERSIAIYLGIGLCLLFIVRTLLLHPAIFGLHHIGMQMRIAMFSLIYKKTLKLSSRVLDKISIGQLVSLLSNNLNKFDEGLALAHFVWIAPLQVALLMGLIWELLQASAFCGLGFLIVLALFQAGLGRMMMKYRDQRAGKISERLVITSEMIENIQSVKAYCWEEAMEKMIENLRQTELKLTRKAAYVRYFNSSAFFFSGFFVVFLSVLPYALIKGIILRKIFTTISFCIVLRMAVTRQFPWAVQTWYDSLGAINKIQDFLQKQEYKTLEYNLTTTEVVMENVTAFWEEGFGELFEKAKQNNNNRKTSNGDDSLFFSNFSLLGTPVLKDINFKIERGQLLAVAGSTGAGKTSLLMVIMGELEPSEGKIKHSGRISFCSQFSWIMPGTIKENIIFGVSYDEYRYRSVIKACQLEEDISKFAEKDNIVLGEGGITLSGGQRARISLARAVYKDADLYLLDSPFGYLDVLTEKEIFESCVCKLMANKTRILVTSKMEHLKKADKILILHEGSSYFYGTFSELQNLQPDFSSKLMGCDSFDQFSAERRNSILTETLHRFSLEGDAPVSWTETKKQSFKQTGEFGEKRKNSILNPINSIRKFSIVQKTPLQMNGIEEDSDEPLERRLSLVPDSEQGEAILPRISVISTGPTLQARRRQSVLNLMTHSVNQGQNIHRKTTASTRKVSLAPQANLTELDIYSRRLSQETGLEISEEINEEDLKECFFDDMESIPAVTTWNTYLRYITVHKSLIFVLIWCLVIFLAEVAASLVVLWLLGNTPLQDKGNSTHSRNNSYAVIITSTSSYYVFYIYVGVADTLLAMGFFRGLPLVHTLITVSKILHHKMLHSVLQAPMSTLNTLKAGGILNRFSKDIAILDDLLPLTIFDFIQLLLIVIGAIAVVAVLQPYIFVATVPVIVAFIMLRAYFLQTSQQLKQLESEGRSPIFTHLVTSLKGLWTLRAFGRQPYFETLFHKALNLHTANWFLYLSTLRWFQMRIEMIFVIFFIAVTFISILTTGEGEGRVGIILTLAMNIMSTLQWAVNSSIDVDSLMRSVSRVFKFIDMPTEGKPTKSTKPYKNGQLSKVMIIENSHVKKDDIWPSGGQMTVKDLTAKYTEGGNAILENISFSISPGQRVGLLGRTGSGKSTLLSAFLRLLNTEGEIQIDGVSWDSITLQQWRKAFGVIPQKVFIFSGTFRKNLDPYEQWSDQEIWKVADEVGLRSVIEQFPGKLDFVLVDGGCVLSHGHKQLMCLARSVLSKAKILLLDEPSAHLDPVTYQIIRRTLKQAFADCTVILCEHRIEAMLECQQFLVIEENKVRQYDSIQKLLNERSLFRQAISPSDRVKLFPHRNSSKCKSKPQIAALKEETEEEVQDTRL

SEQ ID NO: 3 - RNA, 140 nt, Artificial Sequence
  Chemically synthesized oligonucleotides
ggacagaucgccuggagacgccauccacgcuguuuugaccuccauagaagacaccgggaccgauccagccuccgcggccgggaacggugcauuggaacgcggauuccccgugccaagagugacucaccguccuugacacg

SEQ ID NO: 4 - RNA, 105 nt, Artificial Sequence
  Chemically synthesized oligonucleotide
cggguggcaucccugugaccccuccccagugccucuccuggcccuggaaguugccacuccagugcccaccagccuuguccuaauaaaauuaaguugcaucaagcu

SEQ ID NO: 5 - RNA, 105 nt, Artificial Sequence
  Chemically synthesized oligonucleotide
ggguggcaucccugugaccccuccccagugccucuccuggcccuggaaguugccacuccagugcccaccagccuuguccuaauaaaauuaaguugcaucaaagcu

SEQ ID NO: 6 - RNA, 4688 nt, Artificial Sequence
  Chemically synthesized oligonucleotide
ggacagaucgccuggagacgccauccacgcuguuuugaccuccauagaagacaccgggaccgauccagccuccgcggccgggaacggugcauuggaacgcggauuccccgugccaagagugacucaccguccuugacacgaugcaacgcucuccucuugaaaaggccucggugguguccaagcucuucuucucguggacuagacccauccugagaaagggguacagacagcgcuuggagcuguccgauaucuaucaaaucccuuccguggacuccgcggacaaccuguccgagaagcucgagagagaaugggacagagaacucgccucaaagaagaacccgaagcugauuaaugcgcuuaggcggugcuuuuucuggcgguucauguucuacggcaucuuccucuaccugggagaggucaccaaggccgugcagccccuguugcugggacggauuauugccuccuacgaccccgacaacaaggaagaaagaagcaucgcuaucuacuugggcaucggucugugccugcuuuucaucguccggacccucuuguugcauccugcuauuuucggccugcaucacauuggcaugcagaugagaauugccauguuuucccugaucuacaagaaaacucugaagcucucgagccgcgugcuugacaagauuuccaucggccagcucgugucccugcucuccaacaaucugaacaaguucgacgagggccucgcccuggcccacuucguguggaucgccccucugcaaguggcgcuucugaugggccugaucugggagcugcugcaagccucggcauucugugggcuuggauuccugaucgugcuggcacuguuccaggccggacuggggcggaugaugaugaaguacagggaccagagagccggaaagauuuccgaacggcuggugaucacuucggaaaugaucgaaaacauccagucagugaaggccuacugcugggaagaggccauggaaaagaugauugaaaaccuccggcaaaccgagcugaagcugacccgcaaggccgcuuacgugcgcuauuucaacucguccgcuuucuucuucuccggguucuucgugguguuucucuccgugcuccccuacgcccugauuaagggaaucauccucaggaagaucuucaccaccauuuccuucuguaucgugcuccgcauggccgugacccggcaguucccaugggccgugcagacuugguacgacucccugggagccauuaacaagauccaggacuuccuucaaaagcaggaguacaagacccucgaguacaaccugacuacuaccgaggucgugauggaaaacgucaccgccuuuugggaggagggauuuggcgaacuguucgagaaggccaagcagaacaacaacaaccgcaagaccucgaacggugacgacucccucuucuuuucaaacuucagccugcucgggacgcccgugcugaaggacauuaacuucaagaucgaaagaggacagcuccuggcgguggccggaucgaccggagccggaaagacuucccugcugauggugaucaugggagagcuugaaccuagcgagggaaagaucaagcacuccggccgcaucagcuucuguagccaguuuuccuggaucaugcccggaaccauuaaggaaaacaucaucuucggcguguccuacgaugaauaccgcuaccgguccgugaucaaagccugccagcuggaagaggauauuucaaaguucgcggagaaagauaacaucgugcugggcgaaggggguauuaccuugucggggggccagcgggcuagaaucucgcuggccagagccguguauaaggacgccgaccuguaucuccuggacucccccuucggauaccuggacguccugaccgaaaaggagaucuucgaaucgugcgugugcaagcugauggcuaacaagacucgcauccucgugaccuccaaaauggagcaccugaagaaggcagacaagauucugauucugcaugagggguccuccuacuuuuacggcaccuucucggaguugcagaacuugcagcccgacuucucaucgaagcugauggguugcgacagcuucgaccaguucuccgccgaaagaaggaacucgauccugacggaaaccuugcaccgcuucucuuuggaaggcgacgccccugugucauggaccgagacuaagaagcagagcuucaagcagaccggggaauucggcgaaaagaggaagaacagcaucuugaaccccauuaacuccauccgcaaguucucaaucgugcaaaagacgccacugcagaugaacggcauugaggaggacuccgacgaaccccuugagaggcgccugucccuggugccggacagcgagcagggagaagccauccugccucggauuuccgugaucuccacugguccgacgcuccaagcccggcggcggcaguccgugcugaaccugaugacccacagcgugaaccagggccaaaacauucaccgcaagacuaccgcauccacccggaaagugucccuggcaccucaagcgaaucuuaccgagcucgacaucuacucccggagacugucgcaggaaaccgggcucgaaauuuccgaagaaaucaacgaggaggaucugaaagagugcuucuucgacgauauggagucgauacccgccgugacgacuuggaacacuuaucugcgguacaucacugugcacaagucauugaucuucgugcugauuuggugccuggugauuuuccuggccgaggucgcggccucacugguggugcucuggcuguugggaaacacgccucugcaagacaagggaaacuccacgcacucgagaaacaacagcuaugccgugauuaucacuuccaccuccucuuauuacguguucuacaucuacgucggaguggcggauacccugcucgcgauggguuucuucagaggacugccgcugguccacaccuugaucaccgucagcaagauucuucaccacaagauguugcauagcgugcugcaggcccccauguccacccucaacacucugaaggccggaggcauucugaacagauucuccaaggacaucgcuauccuggacgaucuccugccgcuuaccaucuuugacuucauccagcugcugcugaucgugauuggagcaaucgcagugguggcggugcugcagccuuacauuuucguggccacugugccggucauuguggcguucaucaugcugcgggccuacuuccuccaaaccagccagcagcugaagcaacuggaauccgagggacgaucccccaucuucacucaccuugugacgucguugaagggacuguggacccuccgggcuuucggacggcagcccuacuucgaaacccucuuccacaaggcccugaaccuccacaccgccaauugguuccuguaccuguccacccugcggugguuccagaugcgcaucgagaugauuuucgucaucuucuucaucgcggucacauucaucagcauccugacuaccggagagggagagggacgggucggaauaauccugacccucgccaugaacauuaugagcacccugcagugggcagugaacagcucgaucgacguggacagccugaugcgaagcgucagccgcguguucaaguucaucgacaugccuacugagggaaaacccacuaaguccacuaagcccuacaaaaauggccagcugagcaaggucaugaucaucgaaaacucccacgugaagaaggacgauauuuggcccuccggaggucaaaugaccgugaaggaccugaccgcaaaguacaccgagggaggaaacgccauucucgaaaacaucagcuucuccauuucgccgggacagcgggucggccuucucgggcggaccgguuccgggaagucaacucugcugucggcuuuccuccggcugcugaauaccgagggggaaauccaaauugacggcgugucuugggauuccauuacucugcagcaguggcggaaggccuucggcgugaucccccagaagguguucaucuucucggguaccuuccggaagaaccuggauccuuacgagcaguggagcgaccaagaaaucuggaaggucgccgacgaggucggccugcgcuccgugauugaacaauuuccuggaaagcuggacuucgugcucgucgacgggggauguguccugucgcacggacauaagcagcucaugugccucgcacgguccgugcucuccaaggccaagauucugcugcuggacgaaccuucggcccaccuggauccggucaccuaccagaucaucaggaggacccugaagcaggccuuugccgauugcaccgugauucucugcgagcaccgcaucgaggccaugcuggagugccagcaguuccuggucaucgaggagaacaagguccgccaauacgacuccauucaaaagcuccucaacgagcggucgcuguucagacaagcuauuucaccguccgauagagugaagcucuucccgcaucggaacagcucaaagugcaaaucgaagccgcagaucgcagccuugaaggaagagacugaggaagaggugcaggacacccggcuuuaacggguggcaucccugugaccccuccccagugccucuccuggcccuggaaguugccacuccagugcccaccagccuuguccuaauaaaauuaaguugcaucaagcu

SEQ ID NO: 7 - RNA, 4688 nt, Artificial Sequence
  Chemically synthesized oligonucleotide
ggacagaucgccuggagacgccauccacgcuguuuugaccuccauagaagacaccgggaccgauccagccuccgcggccgggaacggugcauuggaacgcggauuccccgugccaagagugacucaccguccuugacacgaugcaacgcucuccucuugaaaaggccucggugguguccaagcucuucuucucguggacuagacccauccugagaaagggguacagacagcgcuuggagcuguccgauaucuaucaaaucccuuccguggacuccgcggacaaccuguccgagaagcucgagagagaaugggacagagaacucgccucaaagaagaacccgaagcugauuaaugcgcuuaggcggugcuuuuucuggcgguucauguucuacggcaucuuccucuaccugggagaggucaccaaggccgugcagccccuguugcugggacggauuauugccuccuacgaccccgacaacaaggaagaaagaagcaucgcuaucuacuugggcaucggucugugccugcuuuucaucguccggacccucuuguugcauccugcuauuuucggccugcaucacauuggcaugcagaugagaauugccauguuuucccugaucuacaagaaaacucugaagcucucgagccgcgugcuugacaagauuuccaucggccagcucgugucccugcucuccaacaaucugaacaaguucgacgagggccucgcccuggcccacuucguguggaucgccccucugcaaguggcgcuucugaugggccugaucugggagcugcugcaagccucggcauucugugggcuuggauuccugaucgugcuggcacuguuccaggccggacuggggcggaugaugaugaaguacagggaccagagagccggaaagauuuccgaacggcuggugaucacuucggaaaugaucgaaaacauccagucagugaaggccuacugcugggaagaggccauggaaaagaugauugaaaaccuccggcaaaccgagcugaagcugacccgcaaggccgcuuacgugcgcuauuucaacucguccgcuuucuucuucuccggguucuucgugguguuucucuccgugcuccccuacgcccugauuaagggaaucauccucaggaagaucuucaccaccauuuccuucuguaucgugcuccgcauggccgugacccggcaguucccaugggccgugcagacuugguacgacucccugggagccauuaacaagauccaggacuuccuucaaaagcaggaguacaagacccucgaguacaaccugacuacuaccgaggucgugauggaaaacgucaccgccuuuugggaggagggauuuggcgaacuguucgagaaggccaagcagaacaacaacaaccgcaagaccucgaacggugacgacucccucuucuuuucaaacuucagccugcucgggacgcccgugcugaaggacauuaacuucaagaucgaaagaggacagcuccuggcgguggccggaucgaccggagccggaaagacuucccugcugauggugaucaugggagagcuugaaccuagcgagggaaagaucaagcacuccggccgcaucagcuucuguagccaguuuuccuggaucaugcccggaaccauuaaggaaaacaucaucuucggcguguccuacgaugaauaccgcuaccgguccgugaucaaagccugccagcuggaagaggauauuucaaaguucgcggagaaagauaacaucgugcugggcgaaggggguauuaccuugucggggggccagcgggcuagaaucucgcuggccagagccguguauaaggacgccgaccuguaucuccuggacucccccuucggauaccuggacguccugaccgaaaaggagaucuucgaaucgugcgugugcaagcugauggcuaacaagacucgcauccucgugaccuccaaaauggagcaccugaagaaggcagacaagauucugauucugcaugagggguccuccuacuuuuacggcaccuucucggaguugcagaacuugcagcccgacuucucaucgaagcugauggguugcgacagcuucgaccaguucuccgccgaaagaaggaacucgauccugacggaaaccuugcaccgcuucucuuuggaaggcgacgccccugugucauggaccgagacuaagaagcagagcuucaagcagaccggggaauucggcgaaaagaggaagaacagcaucuugaaccccauuaacuccauccgcaaguucucaaucgugcaaaagacgccacugcagaugaacggcauugaggaggacuccgacgaaccccuugagaggcgccugucccuggugccggacagcgagcagggagaagccauccugccucggauuuccgugaucuccacugguccgacgcuccaagcccggcggcggcaguccgugcugaaccugaugacccacagcgugaaccagggccaaaacauucaccgcaagacuaccgcauccacccggaaagugucccuggcaccucaagcgaaucuuaccgagcucgacaucuacucccggagacugucgcaggaaaccgggcucgaaauuuccgaagaaaucaacgaggaggaucugaaagagugcuucuucgacgauauggagucgauacccgccgugacgacuuggaacacuuaucugcgguacaucacugugcacaagucauugaucuucgugcugauuuggugccuggugauuuuccuggccgaggucgcggccucacugguggugcucuggcuguugggaaacacgccucugcaagacaagggaaacuccacgcacucgagaaacaacagcuaugccgugauuaucacuuccaccuccucuuauuacguguucuacaucuacgucggaguggcggauacccugcucgcgauggguuucuucagaggacugccgcugguccacaccuugaucaccgucagcaagauucuucaccacaagauguugcauagcgugcugcaggcccccauguccacccucaacacucugaaggccggaggcauucugaacagauucuccaaggacaucgcuauccuggacgaucuccugccgcuuaccaucuuugacuucauccagcugcugcugaucgugauuggagcaaucgcagugguggcggugcugcagccuuacauuuucguggccacugugccggucauuguggcguucaucaugcugcgggccuacuuccuccaaaccagccagcagcugaagcaacuggaauccgagggacgaucccccaucuucacucaccuugugacgucguugaagggacuguggacccuccgggcuuucggacggcagcccuacuucgaaacccucuuccacaaggcccugaaccuccacaccgccaauugguuccuguaccuguccacccugcggugguuccagaugcgcaucgagaugauuuucgucaucuucuucaucgcggucacauucaucagcauccugacuaccggagagggagagggacgggucggaauaauccugacccucgccaugaacauuaugagcacccugcagugggcagugaacagcucgaucgacguggacagccugaugcgaagcgucagccgcguguucaaguucaucgacaugccuacugagggaaaacccacuaaguccacuaagcccuacaaaaauggccagcugagcaaggucaugaucaucgaaaacucccacgugaagaaggacgauauuuggcccuccggaggucaaaugaccgugaaggaccugaccgcaaaguacaccgagggaggaaacgccauucucgaaaacaucagcuucuccauuucgccgggacagcgggucggccuucucgggcggaccgguuccgggaagucaacucugcugucggcuuuccuccggcugcugaauaccgagggggaaauccaaauugacggcgugucuugggauuccauuacucugcagcaguggcggaaggccuucggcgugaucccccagaagguguucaucuucucggguaccuuccggaagaaccuggauccuuacgagcaguggagcgaccaagaaaucuggaaggucgccgacgaggucggccugcgcuccgugauugaacaauuuccuggaaagcuggacuucgugcucgucgacgggggauguguccugucgcacggacauaagcagcucaugugccucgcacgguccgugcucuccaaggccaagauucugcugcuggacgaaccuucggcccaccuggauccggucaccuaccagaucaucaggaggacccugaagcaggccuuugccgauugcaccgugauucucugcgagcaccgcaucgaggccaugcuggagugccagcaguuccuggucaucgaggagaacaagguccgccaauacgacuccauucaaaagcuccucaacgagcggucgcuguucagacaagcuauuucaccguccgauagagugaagcucuucccgcaucggaacagcucaaagugcaaaucgaagccgcagaucgcagccuugaaggaagagacugaggaagaggugcaggacacccggcuuuaaggguggcaucccugugaccccuccccagugccucuccuggcccuggaaguugccacuccagugcccaccagccuuguccuaauaaaauuaaguugcaucaaagcu

SEQ ID NO: 8 - DNA, 4443 bp, Artificial Sequence
  Artificially synthesized oligonucleotide
atgcagaggagcccactggagaaagcctccgtggtgagtaaactcttttttagttggaccagacccatcctgcgaaaaggatacaggcagcgcctcgagttgtcagatatctaccagattccttctgtggactcagctgacaatttgagtgagaagctggagcgggagtgggatagagagctggcgagcaaaaaaaaccccaagcttatcaatgctctgcgccgctgctttttctggaggttcatgttttatgggatcttcctgtacctgggggaggtcaccaaagctgttcagccgctccttcttggccgcatcatcgccagctatgaccctgataataaagaagaaaggtctattgctatttatctgggaattggcctctgcttgctcttcatcgtccgcacccttctgctgcaccctgccatttttggccttcaccacatcggcatgcaaatgagaattgccatgttctccctcatttacaaaaagaccctgaaactttcctcaagagtgttagataaaatatccattggtcagctggtcagcctgctgtccaacaatcttaacaaatttgatgaaggcttggcgctggcccacttcgtgtggattgcacctctgcaggtggccctgttgatgggacttatatgggagctgcttcaagcctctgctttctgtgggctgggctttttgattgtactggcactttttcaggctgggctcggaagaatgatgatgaaatacagagatcagcgggccgggaagatatcagagcgacttgtgatcaccagtgaaatgattgaaaatattcagagcgtgaaagcctactgctgggaagaagccatggagaagatgattgagaacctgaggcagacagagctcaagctcactcggaaggctgcttatgttcgctatttcaacagcagcgccttcttcttcagtggcttctttgttgtcttcctgtctgttctgccatatgcactgataaaaggcattattttacgaaagatcttcaccaccatcagtttttgcatcgttctcaggatggccgtcacaagacagttcccctgggctgtgcagacctggtacgattccttgggggccatcaacaagattcaagatttcttgcaaaaacaagaatataaaactttagaatacaacctcaccaccactgaagtggtcatggaaaatgtgacagccttttgggaggagggttttggagaattgttcgagaaggcaaagcagaataacaacaacaggaagacgagcaatggggacgactctctcttcttcagcaacttttcactgctcgggacccctgtgttgaaagatataaacttcaagatcgagaggggccagctcttggctgtggcaggctccactggagctggtaaaacatctcttctcatggtgatcatgggggaactggagccttccgaaggaaaaatcaagcacagtgggagaatctcattctgcagccagttttcctggatcatgcccggcaccattaaggaaaacatcatatttggagtgtcctatgatgagtaccgctaccggtcagtcatcaaagcctgtcagttggaggaggacatctccaagtttgcagagaaagacaacattgtgcttggagaggggggtatcactctttctggaggacaaagagccaggatctctttggcccgggcagtctacaaggatgcagacctctacttgttggacagtcccttcggctacctcgacgtgctgactgaaaaagaaatttttgaaagctgtgtgtgcaaactgatggcaaacaagaccaggattcttgtcaccagcaagatggaacatctgaagaaagcggacaaaattctgattctgcatgaagggagctcctacttctatggaacatttagcgagcttcagaacctacagccagacttctcctccaaattaatgggctgtgactccttcgaccagttctctgcagaaagaagaaactctatactcacagagaccctccaccgcttctcccttgagggagatgccccagtttcttggacagaaaccaagaagcagtcctttaagcagactggcgagtttggtgaaaagaggaaaaattcaattctcaatccaattaacagtattcgcaagttcagcattgtccagaagacacccctccagatgaatggcatcgaagaagatagtgacgagccgctggagagacggctgagtctggtgccagattcagaacagggggaggccatcctgccccggatcagcgtcatttccacaggccccacattacaagcacggcgccggcagagtgttttaaatctcatgacccattcagtgaaccagggccaaaatatccacaggaagactacagcttctacccggaaagtgtctctggcccctcaggccaatctgaccgagctggacatctacagcaggaggctctcccaggaaacagggctggaaatatctgaagagattaatgaagaggatcttaaagagtgcttctttgatgacatggagagcatccccgcggtgaccacatggaacacctaccttagatatattactgtccacaagagcctcatatttgtcctcatctggtgcctggttattttcctcgctgaggtggcggccagtcttgttgtgctctggctgctgggcaacactcctctccaggacaagggcaatagtactcacagcagaaataattcttatgccgtcatcattacaagcacctccagctactacgtgttctacatctatgtgggcgtggctgacaccctcctggccatgggtttcttccggggcctgcctttggtgcacaccctcatcacagtgtcaaaaattctgcaccataaaatgcttcattctgtcctgcaggcacccatgagcactttgaacacattgaaggctggcggcatcctcaacagattttctaaagatattgctatcctggatgatctcctccccctgacaatctttgactttatccagcttctgctgatcgtgattggagccatagcagtggttgctgtcctgcagccctacatttttgtggccaccgtgcccgtgattgttgcctttattatgctcagagcttacttcctgcaaacttctcaacagctcaaacagctagaatctgagggccggagccccatttttacccacctggtgacttccctgaagggactgtggactctgagagcattcgggcgacagccttactttgagacactgttccacaaggccctgaacttgcacactgccaactggtttctttacctgagcacactccgctggttccagatgcggatagagatgatcttcgtcatcttttttatagctgtaaccttcatttctatccttacaacaggagaaggagagggcagggtgggaatcatcctcacgctggctatgaacataatgtccaccttgcagtgggccgtgaattccagtatagatgtggattctctaatgaggagtgtctcccgggtgtttaaattcattgatatgcctactgaggggaaacccaccaagtcaacaaaaccttataagaatggacagctgagcaaggtgatgataattgagaacagccacgtgaagaaggatgacatttggcccagcgggggccagatgactgtgaaggacctgacggccaagtacaccgaaggtggaaatgccattttggaaaacatcagcttctcaatctctcctgggcagagagttggattgctgggtcgcacgggcagcggcaaatcaaccctgctcagtgccttccttcggctcctgaatacagaaggcgaaatccaaattgacggggtgagctgggacagcatcaccctgcagcagtggagaaaagcatttggggtcattccacagaaagttttcatcttctctggcactttcagaaagaacctggacccctatgagcagtggagcgaccaggagatctggaaggttgcagatgaagttggcctgcggagtgtgatagaacaatttcctggcaagctggattttgtgctggtagatggaggctgcgtgctgtcccacggccacaaacagctgatgtgcctcgcccgctccgttctttcaaaggccaaaatcttgcttttggatgagcccagtgctcacctcgacccagtgacctatcagataatccgcaggaccttaaagcaagcttttgccgactgcaccgtcatactgtgtgagcaccggattgaagcaatgctggaatgccagcagtttctggtgatcgaggagaataaggtccggcagtacgacagcatccagaagttgttgaatgagcgcagccttttccgccaggccatctccccatctgacagagtcaagctgtttccacataggaactcctctaagtgcaagtccaagccccagatcgctgccctcaaggaggaaactgaggaagaggtgcaggatacccgcctgtga

SEQ ID NO: 9 - DNA, 4443 bp, Artificial Sequence
  Chemically synthesized oligonucleotide
atgcagaggagcccactggagaaagcctccgtggtgagtaaactcttttttagttggaccagacccatcctgcgaaaaggatacaggcagcgcctcgagttgtctgatatctaccagattccttctgtggactcagctgacaatttgagtgagaagctggagcgggagtgggatagagagctggcgagcaaaaaaaaccccaagcttatcaatgctctgcgccgctgctttttctggaggttcatgttttatgggatcttcctgtacctgggggaggtcaccaaagctgttcagccgctccttcttggccgcatcatcgccagctatgaccctgataataaagaagaaaggtctattgctatttatctgggaattggcctctgcttgctcttcatcgtccgcacccttctgctgcaccctgccatttttggccttcaccacatcggcatgcaaatgagaattgccatgttctccctcatttacaaaaagaccctgaaactttcctcaagagtgttagataaaatatccattggtcagctggtcagcctgctgtccaacaatcttaacaaatttgatgaaggcttggcgctggcccacttcgtgtggattgcacctctgcaggtggccctgttgatgggacttatatgggagctgcttcaagcctctgctttctgtgggctgggctttttgattgtactggcactttttcaggctgggctcggaagaatgatgatgaaatacagagatcagcgggccgggaagatttcagagcgacttgtgatcaccagtgaaatgattgaaaatattcagagcgtgaaagcctactgctgggaagaagccatggagaagatgattgagaacctgaggcagacagagctcaagctcactcggaaggctgcttatgttcgctatttcaacagcagcgccttcttcttcagtggcttctttgttgtcttcctgtctgttctgccatatgcactgataaaaggcattattttacgaaagatcttcaccaccatcagtttttgcatcgttctcaggatggccgtcacaagacagttcccctgggctgtgcagacctggtacgattccttgggggccatcaacaagattcaagatttcttgcaaaaacaagaatataaaactttagaatacaacctcaccaccactgaagtggtcatggaaaatgtgacagccttttgggaggagggttttggagaattgttcgagaaggcaaagcagaataacaacaacaggaagacgagcaatggggacgactctctcttcttcagcaacttttcactgctcgggacccctgtgttgaaagatataaacttcaagatcgagaggggccagctcttggctgtggcaggctccactggagctggtaaaacatctcttctcatggtgatcatgggggaactggagccttccgaaggaaaaatcaagcacagtgggagaatctcattctgcagccagttttcctggatcatgcccggcaccattaaggaaaacatcatatttggagtgtcctatgatgagtaccgctaccggtcagtcatcaaagcctgtcagttggaggaggacatctccaagtttgcagagaaagacaacattgtgcttggagaggggggtatcactctttctggaggacaaagagccaggatctctttggcccgggcagtctacaaggatgcagacctctacttgttggacagtcccttcggctacctcgacgtgctgactgaaaaagaaatttttgaaagctgtgtgtgcaaactgatggcaaacaagaccaggattcttgtcaccagcaagatggaacatctgaagaaagcggacaaaattctgattctgcatgaagggagctcctacttctatggaacatttagcgagcttcagaacctacagccagacttctcctccaaattaatgggctgtgactccttcgaccagttctctgcagaaagaagaaactctatactcacagagaccctccaccgcttctcccttgagggagatgccccagtttcttggacagaaaccaagaagcagtcctttaagcagactggcgagtttggtgaaaagaggaaaaattcaattctcaatccaattaacagtattcgcaagttcagcattgtccagaagacacccctccagatgaatggcatcgaagaagatagtgacgagccgctggagagacggctgagtctggtgccagattcagaacagggggaggccatcctgccccggatcagcgtcatttccacaggccccacattacaagcacggcgccggcagagtgttttaaatctcatgacccattcagtgaaccagggccaaaatatccacaggaagactacagcttctacccggaaagtgtctctggcccctcaggccaatctgaccgagctggacatctacagcaggaggctctcccaggaaacagggctggaaatatctgaagagattaatgaagaggatcttaaagagtgcttctttgatgacatggagagcatccccgcggtgaccacatggaacacctaccttagatatattactgtccacaagagcctcatatttgtcctcatctggtgcctggttattttcctcgctgaggtggcggccagtcttgttgtgctctggctgctgggcaacactcctctccaggacaagggcaatagtactcacagcagaaataattcttatgccgtcatcattacaagcacctccagctactacgtgttctacatctatgtgggcgtggctgacaccctcctggccatgggtttcttccggggcctgcctttggtgcacaccctcatcacagtgtcaaaaattctgcaccataaaatgcttcattctgtcctgcaggcacccatgagcactttgaacacattgaaggctggcggcatcctcaacagattttctaaagatattgctatcctggatgatctcctccccctgacaatctttgactttatccagcttctgctgatcgtgattggagccatagcagtggttgctgtcctgcagccctacatttttgtggccaccgtgcccgtgattgttgcctttattatgctcagagcttacttcctgcaaacttctcaacagctcaaacagctagaatctgagggccggagccccatttttacccacctggtgacttccctgaagggactgtggactctgagagcattcgggcgacagccttactttgagacactgttccacaaggccctgaacttgcacactgccaactggtttctttacctgagcacactccgctggttccagatgcggatagagatgatcttcgtcatcttttttatagctgtaaccttcatttctatccttacaacaggagaaggagagggcagggtgggaatcatcctcacgctggctatgaacataatgtccaccttgcagtgggccgtgaattccagtatagatgtggattctctaatgaggagtgtctcccgggtgtttaaattcattgatatgcctactgaggggaaacccaccaagtcaacaaaaccttataagaatggacagctgagcaaggtgatgataattgagaacagccacgtgaagaaggatgacatttggcccagcgggggccagatgactgtgaaggacctgacggccaagtacaccgaaggtggaaatgccattttggaaaacatcagcttctcaatctctcctgggcagagagttggattgctgggtcgcacgggcagcggcaaatcaaccctgctcagtgccttccttcggctcctgaatacagaaggcgaaatccaaattgacggggtgagctgggacagcatcaccctgcagcagtggagaaaagcatttggggtcattccacagaaagttttcatcttctctggcactttcagaaagaacctggacccctatgagcagtggagcgaccaggagatctggaaggttgcagatgaagttggcctgcggagtgtgatagaacaatttcctggcaagctggattttgtgctggtagatggaggctgcgtgctgtcccacggccacaaacagctgatgtgcctcgcccgctccgttctttcaaaggccaaaatcttgcttttggatgagcccagtgctcaccttgacccagtgacctatcagataatccgcaggaccttaaagcaagcttttgccgactgcaccgtcatactgtgtgagcaccggattgaagcaatgctggaatgccagcagtttctggtgatcgaggagaataaggtccggcagtacgacagcatccagaagttgttgaatgagcgcagccttttccgccaggccatctccccatctgacagagtcaagctgtttccacataggaactcctctaagtgcaagtccaagccccagatcgctgccctcaaggaggaaactgaggaagaggtgcaggatacccgcctgtga

SEQ ID NO: 10 - DNA, 4443 bp, Artificial Sequence
  Chemically synthesized oligonucleotide
atgcagaggagcccactggagaaagcctccgtggtgagtaaactcttttttagttggaccagacccatcctgcgaaaaggatacaggcagcgcctcgagttgtcagatatctaccagattccttctgtggactcagctgacaatttgagtgagaagctggagcgggagtgggatagagagctggcgagcaaaaaaaaccccaagcttatcaatgctctgcgccgctgctttttctggaggttcatgttttatgggatcttcctgtacctgggggaggtcaccaaagctgttcagccgctccttcttggccgcatcatcgccagctatgaccctgataataaagaagaaaggtctattgctatttatctgggaattggcctctgcttgctcttcatcgtccgcacccttctgctgcaccctgccatttttggccttcaccacatcggcatgcaaatgagaattgccatgttctccctcatttacaaaaagaccctgaaactttcctcaagagtgttagataaaatatccattggtcagctggtcagcctgctgtccaacaatcttaacaaatttgatgaaggcttggcgctggcccacttcgtgtggattgcacctctgcaggtggccctgttgatgggacttatatgggagctgcttcaagcctctgctttctgtgggctgggctttttgattgtactggcactttttcaggctgggctcggaagaatgatgatgaaatacagagatcagcgggccgggaagatatcagagcgacttgtgatcaccagtgaaatgattgaaaatattcagagcgtgaaagcctactgctgggaagaagccatggagaagatgattgagaacctgaggcagacagagctcaagctcactcggaaggctgcttatgttcgctatttcaacagcagcgccttcttcttcagtggcttctttgttgtcttcctgtctgttctgccatatgcactgataaaaggcattattttacgaaagatcttcaccaccatcagtttttgcatcgttctcaggatggccgtcacaagacagttcccctgggctgtgcagacctggtacgattccttgggggccatcaacaagattcaagatttcttgcaaaaacaagaatataaaactttagaatacaacctcaccaccactgaagtggtcatggaaaatgtgacagccttttgggaggagggttttggagaattgttcgagaaggcaaagcagaataacaacaacaggaagacgagcaatggggacgactctctcttcttcagcaacttttcactgctcgggacccctgtgttgaaagatataaacttcaagatcgagaggggccagctcttggctgtggcaggctccactggagctggtaaaacatctcttctcatggtgatcatgggggaactggagccttccgaaggaaaaatcaagcacagtgggagaatctcattctgcagccagttttcctggatcatgcccggcaccattaaggaaaacatcatatttggagtgtcctatgatgagtaccgctaccggtcagtcatcaaagcctgtcagttggaggaggacatctccaagtttgcagagaaagacaacattgtgcttggagaggggggtatcactctttctggaggacaaagagccaggatctctttggcccgggcagtctacaaggatgcagacctctacttgttggacagtcccttcggctacctcgacgtgctgactgaaaaagaaatttttgaaagctgtgtgtgcaaactgatggcaaacaagaccaggattcttgtcaccagcaagatggaacatctgaagaaagcggacaaaattctgattctgcatgaagggagctcctacttctatggaacatttagcgagcttcagaacctacagccagacttctcctccaaattaatgggctgtgactccttcgaccagttctctgcagaaagaagaaactctatactcacagagaccctccaccgcttctcccttgagggagatgccccagtttcttggacagaaaccaagaagcagtcctttaagcagactggcgagtttggtgaaaagaggaaaaattcaattctcaatccaattaacagtattcgcaagttcagcattgtccagaagacacccctccagatgaatggcatcgaagaagatagtgacgagccgctggagagacggctgagtctggtgccagattcagaacagggggaggccatcctgccccggatcagcgtcatttccacaggccccacattacaagcacggcgccggcagagtgttttaaatctcatgacccattcagtgaaccagggccaaaatatccacaggaagactacagcttctacccggaaagtgtctctggcccctcaggccaatctgaccgagctggacatctacagcaggaggctctcccaggaaacagggcttgaaatatctgaagagattaatgaagaggatcttaaagagtgcttctttgatgacatggagagcatccccgcggtgaccacatggaacacctaccttagatatattactgtccacaagagcctcatatttgtcctcatctggtgcctggttattttcctcgctgaggtggcggccagtcttgttgtgctctggctgctgggcaacactcctctccaggacaagggcaatagtacacacagcagaaataattcttatgccgtcatcattacaagcacctccagctactacgtgttctacatctatgtgggcgtggctgacaccctcctggccatgggtttcttccggggcctgcctttggtgcacaccctcatcacagtgtcaaaaattctgcaccataaaatgcttcattctgtcctgcaggcacccatgagcactttgaacacattgaaggctggcggcatcctcaacagattttctaaagatattgctatcctggatgatctcctccccctgacaatctttgactttatccagcttctgctgatcgtgattggagccatagcagtggttgctgtcctgcagccctacatttttgtggccaccgtgcccgtgattgttgcctttattatgctcagagcttacttcctgcaaacttctcaacagctcaaacagctagaatctgagggccggagccccatttttacccacctggtgacttccctgaagggactgtggactctgagagcattcgggcgacagccttactttgagacactgttccacaaggccctgaacttgcacactgccaactggtttctttacctgagcacactccgctggttccagatgcggatagagatgatcttcgtcatcttttttatagctgtaaccttcatttctatccttacaacaggagaaggagagggcagggtgggaatcatcctcacgctggctatgaacataatgtccaccttgcagtgggccgtgaattccagtatagatgtggattctctaatgaggagtgtctcccgggtgtttaaattcattgatatgcctactgaggggaaacccaccaagtcaacaaaaccttataagaatggacagctgagcaaggtgatgataattgagaacagccacgtgaagaaggatgacatttggcccagcgggggccagatgactgtgaaggacctgacggccaagtacaccgaaggtggaaatgccattttggaaaacatcagcttctcaatctctcctgggcagagagttggattgctgggtcgcacgggcagcggcaaatcaaccctgctcagtgccttccttcggctcctgaatacagaaggcgaaatccaaattgacggggtgagctgggacagcatcaccctgcagcagtggagaaaagcatttggggtcattccacagaaagttttcatcttctctggcactttcagaaagaacctggacccctatgagcagtggagcgaccaggagatctggaaggttgcagatgaagttggcctgcggagtgtgatagaacaatttcctggcaagctggattttgtgctggtagatggaggctgcgtgctgtcccacggccacaaacagctgatgtgcctcgcccgctccgttctttcaaaggccaaaatcttgcttttggatgagcccagtgctcaccttgacccagtgacctatcagataatccgcaggaccttaaagcaagcttttgccgactgcaccgtcatactgtgtgagcaccggattgaagcaatgctggaatgccagcagtttctggtgatcgaggagaataaggtccggcagtacgacagcatccagaagttgttgaatgagcgcagccttttccgccaggccatctccccatctgacagagtcaagctgtttccacataggaactcctctaagtgcaagtccaagccccagatcgctgccctcaaggaggaaactgaggaagaggtgcaggatacccgcctgtga

SEQ ID NO: 11 - DNA, 4443 bp, Artificial Sequence
  Chemically synthesized oligonucleotide
atgcagaggagcccactggagaaagcctccgtggtgagtaaactcttttttagttggaccagacccatcctgcgaaaaggatacaggcagcgcctcgagttgtcagatatctaccagattccttctgtggactcagctgacaatttgagtgagaagctggagcgggagtgggatagagagctggcgagcaaaaaaaaccccaagcttatcaatgctctgcgccgctgctttttctggaggttcatgttttatgggatcttcctgtacctgggggaggtcaccaaagctgttcagccgctccttcttggccgcatcatcgccagctatgaccctgataataaagaagaaaggtctattgctatttatctgggaattggcctctgcttgctcttcatcgtccgcacccttctgctgcaccctgccatttttggccttcaccacatcggcatgcaaatgagaattgccatgttctccctcatttacaaaaagaccctgaaactttcctcaagagtgttagataaaatatccattggtcagctggtcagcctgctgtccaacaatcttaacaaatttgatgaaggcttggcgctggcccacttcgtgtggattgcacctctgcaggtggccctgttgatgggacttatatgggagctgcttcaagcctctgctttctgtgggctgggctttttgattgtactggcactttttcaggctgggctcggaagaatgatgatgaaatacagagatcagcgggccgggaagatatcagagcgacttgtgatcaccagtgaaatgattgaaaatattcagagcgtgaaagcctactgctgggaagaagccatggagaagatgattgagaacctgaggcagacagagctcaagctcactcggaaggctgcttatgttcgctatttcaacagcagcgccttcttcttcagtggcttctttgttgtcttcctgtctgttctgccatatgcactgataaaaggcattattttacgaaagatcttcaccaccatcagtttttgcatcgttctcaggatggccgtcacaagacagttcccctgggctgtgcagacctggtacgattccttgggggccatcaacaagattcaagatttcttgcaaaaacaagaatataaaactttagaatacaacctcaccaccactgaagtggtcatggaaaatgtgacagccttttgggaggagggttttggagaattgttcgagaaggcaaagcagaataacaacaacaggaagacgagcaatggggacgactctctcttcttcagcaacttttcactgctcgggacccctgtgttgaaagatataaacttcaagatcgagaggggccagctcttggctgtggcaggctccactggagctggtaaaacatctcttctcatggtgatcatgggggaactggagccttccgaaggaaaaatcaagcacagtgggagaatctcattctgcagccagttttcctggatcatgcccggcaccattaaggaaaacatcatatttggagtgtcctatgatgagtaccgctaccggtcagtcatcaaagcctgtcagttggaggaggacatctccaagtttgcagagaaagacaacattgtgcttggagaggggggtatcactctttctggaggacaaagagccaggatctctttggcccgggcagtctacaaggatgcagacctctacttgttggacagtcccttcggctacctcgacgtgctgactgaaaaagaaatttttgaaagctgtgtgtgcaaactgatggcaaacaagaccaggattcttgtcaccagcaagatggaacatctgaagaaagcggacaaaattctgattctgcatgaagggagctcctacttctatggaacatttagcgagcttcagaacctacagccagacttctcctccaaattaatgggctgtgactccttcgaccagttctctgcagaaagaagaaactctatactcacagagaccctccaccgcttctcccttgagggagatgccccagtttcttggacagaaaccaagaagcagtcctttaagcagactggcgagtttggtgaaaagaggaaaaattcaattctcaatccaattaacagtattcgcaagttcagcattgtccagaagacacccctccagatgaatggcatcgaagaagatagtgacgagccgctggagagacggctgagtctggtgccagattcagaacagggggaggccatcctgccccggatcagcgtcatttccacaggccccacattacaagcacggcgccggcagagtgttttaaatctcatgacccattcagtgaaccagggccaaaatatccacaggaagactacagcttctacccggaaagtgtctctggcccctcaggccaatctgaccgagctggacatctacagcaggaggctctcccaggaaacagggctggaaatatctgaagagattaatgaagaggatcttaaagagtgcttctttgatgacatggagagcatccccgcggtgaccacatggaacacctaccttagatatattactgtccacaagagcctcatatttgtcctcatctggtgcctggttattttcctcgctgaggtggcggccagtcttgttgtgctctggctgctgggcaacactcctctccaggacaagggcaatagtactcacagcagaaataattcttatgccgtcatcattacaagcacctccagctactacgtgttctacatctatgtgggcgtggctgacaccctcctggccatgggtttcttccggggcctgcctttggtgcacaccctcatcacagtgtcaaaaattctgcaccataaaatgcttcattctgtcctgcaggcacccatgagcactttgaacacattgaaggctggcggcatcctcaacagattttctaaagatattgctatcctggatgatctcctccccctgacaatctttgactttatccagcttctgctgatcgtgattggagccatagcagtggttgctgtcctgcagccctacatttttgtggccaccgtgcccgtgattgttgcctttattatgctcagagcttacttcctgcaaacttctcaacagctcaaacagctagaatctgagggccggagccccatttttacccacctggtgacttccctgaagggactgtggactctgagagcattcgggcgacagccttactttgagacactgttccacaaggccctgaacttgcacactgccaactggtttctttacctgagcacactccgctggttccagatgcggatagagatgatcttcgtcatcttttttatagctgtaaccttcatttctatccttacaacaggagaaggagagggcagggtgggaatcatcctcacgctggctatgaacataatgtccaccttgcagtgggccgtgaattccagtatagatgtggattctctaatgaggagtgtctcccgggtgtttaaattcattgatatgccaactgaggggaaacccaccaagtcaacaaaaccttataagaatggacagctgagcaaggtgatgataattgagaacagccacgtgaagaaggatgacatttggcccagcgggggccagatgactgtgaaggacctgacggccaagtacaccgaaggtggaaatgccattttggaaaacatcagcttctcaatctctcctgggcagagagttggattgctgggtcgcacgggcagcggcaaatcaaccctgctcagtgccttccttcggctcctgaatacagaaggcgaaatccaaattgacggggtgagctgggacagcatcaccctgcagcagtggagaaaagcatttggggtcattccacagaaagttttcatcttctctggcactttcagaaagaacctggacccctatgagcagtggagcgaccaggagatctggaaggttgcagatgaagttggcctgcggagtgtgatagaacaatttcctggcaagctggattttgtgctggtagatggaggctgcgtgctgtcccacggccacaaacagctgatgtgcctcgcccgctccgttctttcaaaggccaaaatcttgcttttggatgagcccagtgctcacctcgacccagtgacctatcagataatccgcaggaccttaaagcaagcttttgccgactgcaccgtcatactgtgtgagcaccggattgaagcaatgctggaatgccagcagtttctggtgatcgaggagaataaggtccggcagtacgacagcatccagaagttgttgaatgagcgcagccttttccgccaggccatctccccatctgacagagtcaagctgtttccacataggaactcctctaagtgcaagtccaagccccagatcgctgccctcaaggaggaaactgaggaagaggtgcaggatacccgcctgtga

SEQ ID NO: 12 - DNA, 4443 bp, Artificial Sequence
  Chemically synthesized oligonucleotide
atgcagaggagcccactggagaaagcctccgtggtgagtaaactcttttttagttggaccagacccatcctgcgaaaaggatacaggcagcgcctcgagttgtcagatatctaccagattccttctgtggactcagctgacaatttgagtgagaagctggagcgggagtgggatagagagctggcgagcaaaaaaaaccccaagcttatcaatgctctgcgccgctgctttttctggaggttcatgttttatgggatcttcctgtacctgggggaggtcaccaaagctgttcagccgctccttcttggccgcatcatcgccagctatgaccctgataataaagaagaaaggtctattgctatttatctgggaattggcctctgcttgctcttcatcgtccgcacccttctgctgcaccctgccatttttggccttcaccacatcggcatgcaaatgagaattgccatgttctccctcatttacaaaaagaccctgaaactttcctcaagagtgttagataaaatatccattggtcagctggtcagcctgctgtccaacaatcttaacaaatttgatgaaggcttggcgctggcccacttcgtgtggattgcacctctgcaggtggccctgttgatgggacttatatgggagctgcttcaagcctctgctttctgtgggctgggctttttgattgtactggcactttttcaggctgggctcggaagaatgatgatgaaatacagagatcagcgggccgggaagatatcagagcgacttgtgatcaccagtgaaatgattgaaaatattcagagcgtgaaagcctactgctgggaagaagccatggagaagatgattgagaacctgaggcagacagagctcaagctcactcggaaggctgcttatgttcgctatttcaacagcagcgccttcttcttcagtggcttctttgttgtcttcctgtctgttctgccatatgcactgataaaaggcattattttacgaaagatcttcaccaccatcagtttttgcatcgttctcaggatggccgtcacaagacagttcccctgggctgtgcagacctggtacgattccttgggggccatcaacaagattcaagatttcttgcaaaaacaagaatataaaactttagaatacaacctcaccaccactgaagtggtcatggaaaatgtgacagccttttgggaggagggttttggagaattgttcgagaaggcaaagcagaataacaacaacaggaagacgagcaatggggacgactctctcttcttcagcaacttttcactgctcgggacccctgtgttgaaagatataaacttcaagatcgagaggggccagctcttggctgtggcaggctccactggagctggtaaaacatctcttctcatggtgatcatgggggaactggagccttccgaaggaaaaatcaagcacagtgggagaatctcattctgcagccagttttcctggatcatgcccggcaccattaaggaaaacatcatatttggagtgtcctatgatgagtaccgctaccggtcagtcatcaaagcctgtcagttggaggaggacatctccaagtttgcagagaaagacaacattgtgcttggagaggggggtatcactctttctggaggacaaagagccaggatctctttggcccgggcagtctacaaggatgcagacctctacttgttggacagtcccttcggctacctcgacgtgctgactgaaaaagaaatttttgaaagctgtgtgtgcaaactgatggcaaacaagaccaggattcttgtcaccagcaagatggaacatctgaagaaagcggacaaaattctgattctgcatgaagggagctcctacttctatggaacatttagcgagcttcagaacctacagccagacttctcctccaaattaatgggctgtgactccttcgaccagttctctgcagaaagaagaaactctatactcacagagaccctccaccgcttctcccttgagggagatgccccagtttcttggacagaaaccaagaagcagtcctttaagcagactggcgagtttggtgaaaagaggaaaaattcaattctcaatcctattaacagtattcgcaagttcagcattgtccagaagacacccctccagatgaatggcatcgaagaagatagtgacgagccgctggagagacggctgagtctggtgccagattcagaacagggggaggccatcctgccccggatcagcgtcatttccacaggccccacattacaagcacggcgccggcagagtgttttaaatctcatgacccattcagtgaaccagggccaaaatatccacaggaagactacagcttctacccggaaagtgtctctggcccctcaggccaatctgaccgagctggacatctacagcaggaggctctcccaggaaacagggcttgaaatatctgaagagattaatgaagaggatcttaaagagtgcttctttgatgacatggagagcatccccgcggtgaccacatggaacacctaccttagatatattactgtccacaagagcctcatatttgtcctcatctggtgcctggttattttcctcgctgaggtggcggccagtcttgttgtgctctggctgctgggcaacactcctctccaggacaagggcaatagtactcacagcagaaataattcttatgccgtcatcattacaagcacctccagctactacgtgttctacatctatgtgggcgtggctgacaccctcctggccatgggtttcttccggggcctgcctttggtgcacaccctcatcacagtgtcaaaaattctgcaccataaaatgcttcattctgtcctgcaggcacccatgagcactttgaacacattgaaggctggcggcatcctcaacagattttctaaagatattgctatcctggatgatctcctccccctgacaatctttgactttatccagcttctgctgatcgtgattggagccatagcagtggttgctgtcctgcagccctacatttttgtggccaccgtgcccgtgattgttgcctttattatgctcagagcttacttcctgcaaacttctcaacagctcaaacagctagaatctgagggccggagccccatttttacccacctggtgacttccctgaagggactgtggactctgagagcattcgggcgacagccttactttgagacactgttccacaaggccctgaacttgcacactgccaactggtttctttacctgagcacactccgctggttccagatgcggatagagatgatcttcgtcatcttttttatagctgtaaccttcatttctatccttacaacaggagaaggagagggcagggtgggaatcatcctcacgctggctatgaacataatgtccaccttgcagtgggccgtgaattccagtatagatgtggattctctaatgaggagtgtctcccgggtgtttaaattcattgatatgcctactgaggggaaacccaccaagtcaacaaaaccttataagaatggacagctgagcaaggtgatgataattgagaacagccacgtgaagaaggatgacatttggcccagcgggggccagatgactgtgaaggacctgacggccaagtacaccgaaggtggaaatgccattttggaaaacatcagcttctcaatctctcctgggcagagagttggattgctgggtcgcacgggcagcggcaaatcaaccctgctcagtgccttccttcggctcctgaatacagaaggcgaaatccaaattgacggggtgagctgggacagcatcaccctgcagcagtggagaaaagcatttggggtcattccacagaaagttttcatcttctctggcactttcagaaagaacctggacccctatgagcagtggagcgaccaggagatctggaaggttgcagatgaagttggcctgcggagtgtgatagaacaatttcctggcaagctggattttgtgctggtagatggaggctgcgtgctgtcccacggccacaaacagctgatgtgcctcgcccgctccgttctttcaaaggccaaaatcttgcttttggatgagcccagtgctcacctcgacccagtgacctatcagataatccgcaggaccttaaagcaagcttttgccgactgcaccgtcatactgtgtgagcaccggattgaagcaatgctggaatgccagcagtttctggtgatcgaggagaataaggtccggcagtacgacagcatccagaagttgttgaatgagcgcagccttttccgccaggccatctccccatctgacagagtcaagctgtttccacataggaactcctctaagtgcaagtccaagccccagatcgctgccctcaaggaggaaactgaggaagaggtgcaggatacccgcctgtga

SEQ ID NO: 13 - DNA, 4443 bp, Artificial Sequence
  Chemically synthesized oligonucleotide
atgcagaggagcccactggagaaagcctccgtggtgagtaaactcttttttagttggaccagacccatcctgcgaaaaggatacaggcagcgcctcgagttgtcagatatctaccagattccttctgtggactcagctgacaatttgagtgagaagctggagcgggagtgggatagagagctggcgagcaaaaaaaaccccaagcttatcaatgctctgcgccgctgctttttctggaggttcatgttttatgggatcttcctgtacctgggggaggtcaccaaagctgttcagccgctccttcttggccgcatcatcgccagctatgaccctgataataaagaagaaaggtctattgctatttatctgggaattggcctctgcttgctcttcatcgtccgcacccttctgctgcaccctgccatttttggccttcaccacatcggcatgcaaatgagaattgccatgttctccctcatttacaaaaagaccctgaaactttcctcaagagtgttagataaaatatccattggtcagctggtcagcctgctgtccaacaatcttaacaaatttgatgaaggcttggcgctggcccacttcgtgtggattgcacctctgcaggtggccctgttgatgggacttatatgggagctgcttcaagcctctgctttctgtgggctgggctttttgattgtactggcactttttcaggctgggctcggaagaatgatgatgaaatacagagatcagcgggccgggaagatttcagagcgacttgtgatcaccagtgaaatgattgaaaatattcagagcgtgaaagcctactgctgggaagaagccatggagaagatgattgagaacctgaggcagacagagctcaagctcactcggaaggctgcttatgttcgctatttcaacagcagcgccttcttcttcagtggcttctttgttgtcttcctgtctgttctgccatatgcactgataaaaggcattattttacgaaagatcttcaccaccatcagtttttgcatcgttctcaggatggccgtcacaagacagttcccctgggctgtgcagacctggtacgattccttgggggccatcaacaagattcaagatttcttgcaaaaacaagaatataaaactttagaatacaacctcaccaccactgaagtggtcatggaaaatgtgacagccttttgggaggagggttttggagaattgttcgagaaggcaaagcagaataacaacaacaggaagacgagcaatggggacgactctctcttcttcagcaacttttcactgctcgggacccctgtgttgaaagatataaacttcaagatcgagaggggccagctcttggctgtggcaggctccactggagctggtaaaacatctcttctcatggtgatcatgggggaactggagccttccgaaggaaaaatcaagcacagtgggagaatctcattctgcagccagttttcctggatcatgcccggcaccattaaggaaaacatcatatttggagtgtcctatgatgagtaccgctaccggtcagtcatcaaagcctgtcagttggaggaggacatctccaagtttgcagagaaagacaacattgtgcttggagaggggggtatcactctttctggaggacaaagagccaggatctctttggcccgggcagtctacaaggatgcagacctctacttgttggacagtcccttcggctacctcgacgtgctgactgaaaaagaaatttttgaaagctgtgtgtgcaaactgatggcaaacaagaccaggattcttgtcaccagcaagatggaacatctgaagaaagcggacaaaattctgattctgcatgaagggagctcctacttctatggaacatttagcgagcttcagaacctacagccagacttctcctccaaattaatgggctgtgactccttcgaccagttctctgcagaaagaagaaactctatactcacagagaccctccaccgcttctcccttgagggagatgccccagtttcttggacagaaaccaagaagcagtcctttaagcagactggcgagtttggtgaaaagaggaaaaattcaattctcaatccaattaacagtattcgcaagttcagcattgtccagaagacacccctccagatgaatggcatcgaagaagatagtgacgagccgctggagagacggctgagtctggtgccagattcagaacagggggaggccatcctgccccggatcagcgtcatttccacaggccccacattacaagcacggcgccggcagagtgttttaaatctcatgacccattcagtgaaccagggccaaaatatccacaggaagactacagcttctacccggaaagtgtctctggcccctcaggccaatctgaccgagctggacatctacagcaggaggctctcccaggaaacagggctggaaatatctgaagagattaatgaagaggatcttaaagagtgcttctttgatgacatggagagcatccccgcggtgaccacatggaacacctaccttagatatattactgtccacaagagcctcatatttgtcctcatctggtgcctggttattttcctcgctgaggtggcggccagtcttgttgtgctctggctgctgggcaacactcctctccaggacaagggcaatagtactcacagcagaaataattcttatgccgtcatcattacaagcacctccagctactacgtgttctacatctatgtgggcgtggctgacaccctcctggccatgggtttcttccggggcctgcctttggtgcacaccctcatcacagtgtcaaaaattctgcaccataaaatgcttcattctgtcctgcaggcacccatgagcactttgaacacattgaaggctggcggcatcctcaacagattttctaaagatattgctatcctggatgatctcctccccctgacaatctttgactttatccagcttctgctgatcgtgattggagccatagcagtggttgctgtcctgcagccctacatttttgtggccaccgtgcccgtgattgttgcctttattatgctcagagcttacttcctgcaaacttctcaacagctcaaacagctagaatctgagggccggagccccatttttacccacctggtgacttccctgaagggactgtggactctgagagcattcgggcgacagccttactttgagacactgttccacaaggccctgaacttgcacactgccaactggtttctttacctgagcacactccgctggttccagatgcggatagagatgatcttcgtcatcttttttatagctgtaaccttcatttctatccttacaacaggagaaggagagggcagggtgggaatcatcctcacgctggctatgaacataatgtccaccttgcagtgggccgtgaattccagtatagatgtggattctctaatgaggagtgtctcccgggtgtttaaattcattgatatgccaactgaggggaaacccaccaagtcaacaaaaccttataagaatggacagctgagcaaggtgatgataattgagaacagccacgtgaagaaggatgacatttggcccagcgggggccagatgactgtgaaggacctgacggccaagtacaccgaaggtggaaatgccattttggaaaacatcagcttctcaatctctcctgggcagagagttggattgctgggtcgcacgggcagcggcaaatcaaccctgctcagtgccttccttcggctcctgaatacagaaggcgaaatccaaattgacggggtgagctgggacagcatcaccctgcagcagtggagaaaagcatttggggtcattccacagaaagttttcatcttctctggcactttcagaaagaacctggacccctatgagcagtggagcgaccaggagatctggaaggttgcagatgaagttggcctgcggagtgtgatagaacaatttcctggcaagctggattttgtgctggtagatggaggctgcgtgctgtcccacggccacaaacagctgatgtgcctcgcccgctccgttctttcaaaggccaaaatcttgcttttggatgagcccagtgctcacctcgacccagtgacctatcagataatccgcaggaccttaaagcaagcttttgccgactgcaccgtcatactgtgtgagcaccggattgaagcaatgctggaatgccagcagtttctggtgatcgaggagaataaggtccggcagtacgacagcatccagaagttgttgaatgagcgcagccttttccgccaggccatctccccatctgacagagtcaagctgtttccacataggaactcctctaagtgcaagtccaagccccagatcgctgccctcaaggaggaaactgaggaagaggtgcaggatacccgcctgtga

SEQ ID NO: 14 - DNA, 4443 bp, Artificial Sequence
  Chemically synthesized oligonucleotide
atgcagaggagcccactggagaaagcctccgtggtgagtaaactcttttttagttggaccagacccatcctgcgaaaaggatacaggcagcgcctcgagttgtctgatatctaccagattccttctgtggactcagctgacaatttgagtgagaagctggagcgggagtgggatagagagctggcgagcaaaaaaaaccccaagcttatcaatgctctgcgccgctgctttttctggaggttcatgttttatgggatcttcctgtacctgggggaggtcaccaaagctgttcagccgctccttcttggccgcatcatcgccagctatgaccctgataataaagaagaaaggtctattgctatttatctgggaattggcctctgcttgctcttcatcgtccgcacccttctgctgcaccctgccatttttggccttcaccacatcggcatgcaaatgagaattgccatgttctccctcatttacaaaaagaccctgaaactttcctcaagagtgttagataaaatatccattggtcagctggtcagcctgctgtccaacaatcttaacaaatttgatgaaggcttggcgctggcccacttcgtgtggattgcacctctgcaggtggccctgttgatgggacttatatgggagctgcttcaagcctctgctttctgtgggctgggctttttgattgtactggcactttttcaggctgggctcggaagaatgatgatgaaatacagagatcagcgggccgggaagatatcagagcgacttgtgatcaccagtgaaatgattgaaaatattcagagcgtgaaagcctactgctgggaagaagccatggagaagatgattgagaacctgaggcagacagagctcaagctcactcggaaggctgcttatgttcgctatttcaacagcagcgccttcttcttcagtggcttctttgttgtcttcctgtctgttctgccatatgcactgataaaaggcattattttacgaaagatcttcaccaccatcagtttttgcatcgttctcaggatggccgtcacaagacagttcccctgggctgtgcagacctggtacgattccttgggggccatcaacaagattcaagatttcttgcaaaaacaagaatataaaactttagaatacaacctcaccaccactgaagtggtcatggaaaatgtgacagccttttgggaggagggttttggagaattgttcgagaaggcaaagcagaataacaacaacaggaagacgagcaatggggacgactctctcttcttcagcaacttttcactgctcgggacccctgtgttgaaagatataaacttcaagatcgagaggggccagctcttggctgtggcaggctccactggagctggtaaaacatctcttctcatggtgatcatgggggaactggagccttccgaaggaaaaatcaagcacagtgggagaatctcattctgcagccagttttcctggatcatgcccggcaccattaaggaaaacatcatatttggagtgtcctatgatgagtaccgctaccggtccgtcatcaaagcctgtcagttggaggaggacatctccaagtttgcagagaaagacaacattgtgcttggagaggggggtatcactctttctggaggacaaagagccaggatctctttggcccgggcagtctacaaggatgcagacctctacttgttggacagtcccttcggctacctcgacgtgctgactgaaaaagaaatttttgaaagctgtgtgtgcaaactgatggcaaacaagaccaggattcttgtcaccagcaagatggaacatctgaagaaagcggacaaaattctgattctgcatgaagggagctcctacttctatggaacatttagcgagcttcagaacctacagccagacttctcctccaaattaatgggctgtgactccttcgaccagttctctgcagaaagaagaaactctatactcacagagaccctccaccgcttctcccttgagggagatgccccagtttcttggacagaaaccaagaagcagtcctttaagcagactggcgagtttggtgaaaagaggaaaaattcaattctcaatccaattaacagtattcgcaagttcagcattgtccagaagacacccctccagatgaatggcatcgaagaagatagtgacgagccgctggagagacggctgagtctggtgccagattcagaacagggggaggccatcctgccccggatcagcgtcatttccacaggccccacattacaagcacggcgccggcagagtgttttaaatctcatgacccattcagtgaaccagggccaaaatatccacaggaagactacagcttctacccggaaagtgtctctggcccctcaggccaatctgaccgagctggacatctacagcaggaggctctcccaggaaacagggcttgaaatatctgaagagattaatgaagaggatcttaaagagtgcttctttgatgacatggagagcatccccgcggtgaccacatggaacacctaccttagatatattactgtccacaagagcctcatatttgtcctcatctggtgcctggttattttcctcgctgaggtggcggccagtcttgttgtgctctggctgctgggcaacactcctctccaggacaagggcaatagtactcacagcagaaataattcttatgccgtcatcattacaagcacctccagctactacgtgttctacatctatgtgggcgtggctgacaccctcctggccatgggtttcttccggggcctgcctttggtgcacaccctcatcacagtgtcaaaaattctgcaccataaaatgcttcattctgtcctgcaggcacccatgagcactttgaacacattgaaggctggcggcatcctcaacagattttctaaagatattgctatcctggatgatctcctccccctgacaatctttgactttatccagcttctgctgatcgtgattggagccatagcagtggttgctgtcctgcagccctacatttttgtggccaccgtgcccgtgattgttgcctttattatgctcagagcttacttcctgcaaacttctcaacagctcaaacagctagaatctgagggccggagccccatttttacccacctggtgacttccctgaagggactgtggactctgagagcattcgggcgacagccttactttgagacactgttccacaaggccctgaacttgcacactgccaactggtttctttacctgagcacactccgctggttccagatgcggatagagatgatcttcgtcatcttttttatagctgtaaccttcatttctatccttacaacaggagaaggagagggcagggtgggaatcatcctcacgctggctatgaacataatgtccaccttgcagtgggccgtgaattccagtatagatgtggattctctaatgaggagtgtctcccgggtgtttaaattcattgatatgcctactgaggggaaacccaccaagtcaacaaagccttataagaatggacagctgagcaaggtgatgataattgagaacagccacgtgaagaaggatgacatttggcccagcgggggccagatgactgtgaaggacctgacggccaagtacaccgaaggtggaaatgccattttggaaaacatcagcttctcaatctctcctgggcagagagttggattgctgggtcgcacgggcagcggcaaatcaaccctgctcagtgccttccttcggctcctgaatacagaaggcgaaatccaaattgacggggtgagctgggacagcatcaccctgcagcagtggagaaaagcatttggggtcattccacagaaagttttcatcttctctggcactttcagaaagaacctggacccctatgagcagtggagcgaccaggagatctggaaggttgcagatgaagttggcctgcggagtgtgatagaacaatttcctggcaagctggattttgtgctggtagatggaggctgcgtgctgtcccacggccacaaacagctgatgtgcctcgcccgctccgttctttcaaaggccaaaatcttgcttttggatgagcccagtgctcacctcgacccagtgacctatcagataatccgcaggaccttaaagcaagcttttgccgactgcaccgtcatactgtgtgagcaccggattgaagcaatgctggaatgccagcagtttctggtgatcgaggagaataaggtccggcagtacgacagcatccagaagttgttgaatgagcgcagccttttccgccaggccatctccccatctgacagagtcaagctgtttccacataggaactcctctaagtgcaagtccaagccccagatcgctgccctcaaggaggaaactgaggaagaggtgcaggatacccgcctgtga

SEQ ID NO: 15 - DNA, 4443 bp, Artificial Sequence
  Chemically synthesized oligonucleotide
atgcagaggagcccactggagaaagcctccgtggtgagtaaactcttttttagttggaccagacccatcctgcgaaaaggatacaggcagcgcctcgagttgtcagatatctaccagattccttctgtggactcagctgacaatttgagtgagaagctggagcgggagtgggatagagagctggcgagcaaaaaaaaccccaagcttatcaatgctctgcgccgctgctttttctggaggttcatgttttatgggatcttcctgtacctgggggaggtcaccaaagctgttcagccgctccttcttggccgcatcatcgccagctatgaccctgataataaagaagaaaggtctattgctatttatctgggaattggcctctgcttgctcttcatcgtccgcacccttctgctgcaccctgccatttttggccttcaccacatcggcatgcaaatgagaattgccatgttctccctcatttacaaaaagaccctgaaactttcctcaagagtgttagataaaatatccattggtcagctggtcagcctgctgtccaacaatcttaacaaatttgatgaaggcttggcgctggcccacttcgtgtggattgcacctctgcaggtggccctgttgatgggacttatatgggagctgcttcaagcctctgctttctgtgggctgggctttttgattgtactggcactttttcaggctgggctcggaagaatgatgatgaaatacagagatcagcgggccgggaagatatcagagcgacttgtgatcaccagtgaaatgattgaaaatattcagagcgtgaaagcctactgctgggaagaagccatggagaagatgattgagaacctgaggcagacagagctcaagctcactcggaaggctgcttatgttcgctatttcaacagcagcgccttcttcttcagtggcttctttgttgtcttcctgtctgttctgccatatgcactgataaaaggcattattttacgaaagatcttcaccaccatcagtttttgcatcgttctcaggatggccgtcacaagacagttcccctgggctgtgcagacctggtacgattccttgggggccatcaacaagattcaagatttcttgcaaaaacaagaatataaaactttagaatacaacctcaccaccactgaagtggtcatggaaaatgtgacagccttttgggaggagggttttggagaattgttcgagaaggcaaagcagaataacaacaacaggaagacgagcaatggggacgactctctcttcttcagcaacttttcactgctcgggacccctgtgttgaaagatataaacttcaagatcgagaggggccagctcttggctgtggcaggctccactggagctggtaaaacatctcttctcatggtgatcatgggggaactggagccttccgaaggaaaaatcaagcacagtgggagaatctcattctgcagccagttttcctggatcatgcccggcaccattaaggaaaacatcatatttggagtgtcctatgatgagtaccgctaccggtcagtcatcaaagcctgtcagttggaggaggacatctccaagtttgcagagaaagacaacattgtgcttggagaggggggtatcactctttctggaggacaaagagccaggatctctttggcccgggcagtctacaaggatgcagacctctacttgttggacagtcccttcggctacctcgacgtgctgactgaaaaagaaatttttgaaagctgtgtgtgcaaactgatggcaaacaagaccaggattcttgtcaccagcaagatggaacatctgaagaaagcggacaaaattctgattctgcatgaagggagctcctacttctatggaacatttagcgagcttcagaacctacagccagacttctcctccaaattaatgggctgtgactccttcgaccagttctctgcagaaagaagaaactctatactcacagagaccctccaccgcttctcccttgagggagatgccccagtttcttggacagaaaccaagaagcagtcctttaagcagactggcgagtttggtgaaaagaggaaaaattcaattctcaatcctattaacagtattcgcaagttcagcattgtccagaagacacccctccagatgaatggcatcgaagaagatagtgacgagccgctggagagacggctgagtctggtgccagattcagaacagggggaggccatcctgccccggatcagcgtcatttccacaggccccacattacaagcacggcgccggcagagtgttttaaatctcatgacccattcagtgaaccagggccaaaatatccacaggaagactacagcttctacccggaaagtgtctctggcccctcaggccaatctgaccgagctggacatctacagcaggaggctctcccaggaaacagggcttgaaatatctgaagagattaatgaagaggatcttaaagagtgcttctttgatgacatggagagcatccccgcggtgaccacatggaacacctaccttagatatattactgtccacaagagcctcatatttgtcctcatctggtgcctggttattttcctcgctgaggtggcggccagtcttgttgtgctctggctgctgggcaacactcctctccaggacaagggcaatagtacacacagcagaaataattcttatgccgtcatcattacaagcacctccagctactacgtgttctacatctatgtgggcgtggctgacaccctcctggccatgggtttcttccggggcctgcctttggtgcacaccctcatcacagtgtcaaaaattctgcaccataaaatgcttcattctgtcctgcaggcacccatgagcactttgaacacattgaaggctggcggcatcctcaacagattttctaaagatattgctatcctggatgatctcctccccctgacaatctttgactttatccagcttctgctgatcgtgattggagccatagcagtggttgctgtcctgcagccctacatttttgtggccaccgtgcccgtgattgttgcctttattatgctcagagcttacttcctgcaaacttctcaacagctcaaacagctagaatctgagggccggagccccatttttacccacctggtgacttccctgaagggactgtggactctgagagcattcgggcgacagccttactttgagacactgttccacaaggccctgaacttgcacactgccaactggtttctttacctgagcacactccgctggttccagatgcggatagagatgatcttcgtcatcttttttatagctgtaaccttcatttctatccttacaacaggagaaggagagggcagggtgggaatcatcctcacgctggctatgaacataatgtccaccttgcagtgggccgtgaattccagtatagatgtggattctctaatgaggagtgtctcccgggtgtttaaattcattgatatgcctactgaggggaaacccaccaagtcaacaaaaccttataagaatggacagctgagcaaggtgatgataattgagaacagccacgtgaagaaggatgacatttggcccagcgggggccagatgactgtgaaggacctgacggccaagtacaccgaaggtggaaatgccattttggaaaacatcagcttctcaatctctcctgggcagagagttggattgctgggtcgcacgggcagcggcaaatcaaccctgctcagtgccttccttcggctcctgaatacagaaggcgaaatccaaattgacggggtgagctgggacagcatcaccctgcagcagtggagaaaagcatttggggtcattccacagaaagttttcatcttctctggcactttcagaaagaacctggacccctatgagcagtggagcgaccaggagatctggaaggttgcagatgaagttggcctgcggagtgtgatagaacaatttcctggcaagctggattttgtgctggtagatggaggctgcgtgctgtcccacggccacaaacagctgatgtgcctcgcccgctccgttctttcaaaggccaaaatcttgcttttggatgagcccagtgctcacctcgacccagtgacctatcagataatccgcaggaccttaaagcaagcttttgccgactgcaccgtcatactgtgtgagcaccggattgaagcaatgctggaatgccagcagtttctggtgatcgaggagaataaggtccggcagtacgacagcatccagaagttgttgaatgagcgcagccttttccgccaggccatctccccatctgacagagtcaagctgtttccacataggaactcctctaagtgcaagtccaagccccagatcgctgccctcaaggaggaaactgaggaagaggtgcaggatacccgcctgtga

SEQ ID NO: 16 - DNA, 4443 bp, Artificial Sequence
  Chemically synthesized oligonucleotide
atgcagaggagcccactggagaaagcctccgtggtgagtaaactcttttttagttggaccagacccatcctgcgaaaaggatacaggcagcgcctcgagttgtcagatatctaccagattccttctgtggactcagctgacaatttgagtgagaagctggagcgggagtgggatagagagctggcgagcaaaaaaaaccccaagcttatcaatgctctgcgccgctgctttttctggaggttcatgttttatgggatcttcctgtacctgggggaggtcaccaaagctgttcagccgctccttcttggccgcatcatcgccagctatgaccctgataataaagaagaaaggtctattgctatttatctgggaattggcctctgcttgctcttcatcgtccgcacccttctgctgcaccctgccatttttggccttcaccacatcggcatgcaaatgagaattgccatgttctccctcatttacaaaaagaccctgaaactttcctcaagagtgttagataaaatatccattggtcagctggtcagcctgctgtccaacaatcttaacaaatttgatgaaggcttggcgctggcccacttcgtgtggattgcacctctgcaggtggccctgttgatgggacttatatgggagctgcttcaagcctctgctttctgtgggctgggctttttgattgtactggcactttttcaggctgggctcggaagaatgatgatgaaatacagagatcagcgggccgggaagatatcagagcgacttgtgatcaccagtgaaatgattgaaaatattcagagcgtgaaagcctactgctgggaagaagccatggagaagatgattgagaacctgaggcagacagagctcaagctcactcggaaggctgcttatgttcgctatttcaacagcagcgccttcttcttcagtggcttctttgttgtcttcctgtctgttctgccatatgcactgataaaaggcattattttacgaaagatcttcaccaccatcagtttttgcatcgttctcaggatggccgtcacaagacagttcccctgggctgtgcagacctggtacgattccttgggggccatcaacaagattcaagatttcttgcaaaaacaagaatataaaactttagaatacaacctcaccaccactgaagtggtcatggaaaatgtgacagccttttgggaggagggttttggagaattgttcgagaaggcaaagcagaataacaacaacaggaagacgagcaatggggacgactctctcttcttcagcaacttttcactgctcgggacccctgtgttgaaagatataaacttcaagatcgagaggggccagctcttggctgtggcaggctccactggagctggtaaaacatctcttctcatggtgatcatgggggaactggagccttccgaaggaaaaatcaagcacagtgggagaatctcattctgcagccagttttcctggatcatgcccggcaccattaaggaaaacatcatatttggagtgtcctatgatgagtaccgctaccggtccgtcatcaaagcctgtcagttggaggaggacatctccaagtttgcagagaaagacaacattgtgcttggagaggggggtatcactctttctggaggacaaagagccaggatctctttggcccgggcagtctacaaggatgcagacctctacttgttggacagtcccttcggctacctcgacgtgctgactgaaaaagaaatttttgaaagctgtgtgtgcaaactgatggcaaacaagaccaggattcttgtcaccagcaagatggaacatctgaagaaagcggacaaaattctgattctgcatgaagggagctcctacttctatggaacatttagcgagcttcagaacctacagccagacttctcctccaaattaatgggctgtgactccttcgaccagttctctgcagaaagaagaaactctatactcacagagaccctccaccgcttctcccttgagggagatgccccagtttcttggacagaaaccaagaagcagtcctttaagcagactggcgagtttggtgaaaagaggaaaaattcaattctcaatccaattaacagtattcgcaagttcagcattgtccagaagacacccctccagatgaatggcatcgaagaagatagtgacgagccgctggagagacggctgagtctggtgccagattcagaacagggggaggccatcctgccccggatcagcgtcatttccacaggccccacattacaagcacggcgccggcagagtgttttaaatctcatgacccattcagtgaaccagggccaaaatatccacaggaagactacagcttctacccggaaagtgtctctggcccctcaggccaatctgaccgagctggacatctacagcaggaggctctcccaggaaacagggctggaaatatctgaagagattaatgaagaggatcttaaagagtgcttctttgatgacatggagagcatccccgcggtgaccacatggaacacctaccttagatatattactgtccacaagagcctcatatttgtcctcatctggtgcctggttattttcctcgctgaggtggcggccagtcttgttgtgctctggctgctgggcaacactcctctccaggacaagggcaatagtactcacagcagaaataattcttatgccgtcatcattacaagcacctccagctactacgtgttctacatctatgtgggcgtggctgacaccctcctggccatgggtttcttccggggcctgcctttggtgcacaccctcatcacagtgtcaaaaattctgcaccataaaatgcttcattctgtcctgcaggcacccatgagcactttgaacacattgaaggctggcggcatcctcaacagattttctaaagatattgctatcctggatgatctcctccccctgacaatctttgactttatccagcttctgctgatcgtgattggagccatagcagtggttgctgtcctgcagccctacatttttgtggccaccgtgcccgtgattgttgcctttattatgctcagagcttacttcctgcaaacttctcaacagctcaaacagctagagtctgagggccggagccccatttttacccacctggtgacttccctgaagggactgtggactctgagagcattcgggcgacagccttactttgagacactgttccacaaggccctgaacttgcacactgccaactggtttctttacctgagcacactccgctggttccagatgcggatagagatgatcttcgtcatcttttttatagctgtaaccttcatttctatccttacaacaggagaaggagagggcagggtgggaatcatcctcacgctggctatgaacataatgtccaccttgcagtgggccgtgaattccagtatagatgtggattctctaatgaggagtgtctcccgggtgtttaaattcattgatatgcctactgaggggaaacccaccaagtcaacaaaaccttataagaatggacagctgagcaaggtgatgataattgagaacagccacgtgaagaaggatgacatttggcccagcgggggccagatgactgtgaaggacctgacggccaagtacaccgaaggtggaaatgccattttggaaaacatcagcttctcaatctctcctgggcagagagttggattgctgggtcgcacgggcagcggcaaatcaaccctgctcagtgccttccttcggctcctgaatacagaaggcgaaatccaaattgacggggtgagctgggacagcatcaccctgcagcagtggagaaaagcatttggggtcattccacagaaagttttcatcttctctggcactttcagaaagaacctggacccctatgagcagtggagcgaccaggagatctggaaggttgcagatgaagttggcctgcggagtgtgatagaacaatttcctggcaagctggattttgtgctggtagatggaggctgcgtgctgtcccacggccacaaacagctgatgtgcctcgcccgctccgttctttcaaaggccaaaatcttgcttttggatgagcccagtgctcacctcgacccagtgacctatcagataatccgcaggaccttaaagcaagcttttgccgactgcaccgtcatactgtgtgagcaccggattgaagcaatgctggaatgccagcagtttctggtgatcgaggagaataaggtccggcagtacgacagcatccagaagttgttgaatgagcgcagccttttccgccaggccatctccccatctgacagagtcaagctgtttccacataggaactcctctaagtgcaagtccaagccccagatcgctgccctcaaggaggaaactgaggaagaggtgcaggatacccgcctgtga

SEQ ID NO: 17 - DNA, 4443 bp, Artificial Sequence
  Chemically synthesized oligonucleotide
atgcagaggagcccactggagaaagcctccgtggtgagtaaactcttttttagttggaccagacccatcctgcgaaaaggatacaggcagcgcctcgagttgtctgatatctaccagattccttctgtggactcagctgacaatttgagtgagaagctggagcgggagtgggatagagagctggcgagcaaaaaaaaccccaagcttatcaatgctctgcgccgctgctttttctggaggttcatgttttatgggatcttcctgtacctgggggaggtcaccaaagctgttcagccgctccttcttggccgcatcatcgccagctatgaccctgataataaagaagaaaggtctattgctatttatctgggaattggcctctgcttgctcttcatcgtccgcacccttctgctgcaccctgccatttttggccttcaccacatcggcatgcaaatgagaattgccatgttctccctcatttacaaaaagaccctgaaactttcctcaagagtgttagataaaatatccattggtcagctggtcagcctgctgtccaacaatcttaacaaatttgatgaaggcttggcgctggcccacttcgtgtggattgcacctctgcaggtggccctgttgatgggacttatatgggagctgcttcaagcctctgctttctgtgggctgggctttttgattgtactggcactttttcaggctgggctcggaagaatgatgatgaaatacagagatcagcgggccgggaagatttcagagcgacttgtgatcaccagtgaaatgattgaaaatattcagagcgtgaaagcctactgctgggaagaagccatggagaagatgattgagaacctgaggcagacagagctcaagctcactcggaaggctgcttatgttcgctatttcaacagcagcgccttcttcttcagtggcttctttgttgtcttcctgtctgttctgccatatgcactgataaaaggcattattttacgaaagatcttcaccaccatcagtttttgcatcgttctcaggatggccgtcacaagacagttcccctgggctgtgcagacctggtacgattccttgggggccatcaacaagattcaagatttcttgcaaaaacaagaatataaaactttagaatacaacctcaccaccactgaagtggtcatggaaaatgtgacagccttttgggaggagggttttggagaattgttcgagaaggcaaagcagaataacaacaacaggaagacgagcaatggggacgactctctcttcttcagcaacttttcactgctcgggacccctgtgttgaaagatataaacttcaagatcgagaggggccagctcttggctgtggcaggctccactggagctggtaaaacatctcttctcatggtgatcatgggggaactggagccttccgaaggaaaaatcaagcacagtgggagaatctcattctgcagccagttttcctggatcatgcccggcaccattaaggaaaacatcatatttggagtgtcctatgatgagtaccgctaccggtcagtcatcaaagcctgtcagttggaggaggacatctccaagtttgcagagaaagacaacattgtgcttggagaggggggtatcactctttctggaggacaaagagccaggatctctttggcccgggcagtctacaaggatgcagacctctacttgttggacagtcccttcggctacctcgacgtgctgactgaaaaagaaatttttgaaagctgtgtgtgcaaactgatggcaaacaagaccaggattcttgtcaccagcaagatggaacatctgaagaaagcggacaaaattctgattctgcatgaagggagctcctacttctatggaacatttagcgagcttcagaacctacagccagacttctcctccaaattaatgggctgtgactccttcgaccagttctctgcagaaagaagaaactctatactcacagagaccctccaccgcttctcccttgagggagatgccccagtttcttggacagaaaccaagaagcagtcctttaagcagactggcgagtttggtgaaaagaggaaaaattcaattctcaatcctattaacagtattcgcaagttcagcattgtccagaagacacccctccagatgaatggcatcgaagaagatagtgacgagccgctggagagacggctgagtctggtgccagattcagaacagggggaggccatcctgccccggatcagcgtcatttccacaggccccacattacaagcacggcgccggcagagtgttttaaatctcatgacccattcagtgaaccagggccaaaatatccacaggaagactacagcttctacccggaaagtgtctctggcccctcaggccaatctgaccgagctggacatctacagcaggaggctctcccaggaaacagggctggaaatatctgaagagattaatgaagaggatcttaaagagtgcttctttgatgacatggagagcatccccgcggtgaccacatggaacacctaccttagatatattactgtccacaagagcctcatatttgtcctcatctggtgcctggttattttcctcgctgaggtggcggccagtcttgttgtgctctggctgctgggcaacactcctctccaggacaagggcaatagtacacacagcagaaataattcttatgccgtcatcattacaagcacctccagctactacgtgttctacatctatgtgggcgtggctgacaccctcctggccatgggtttcttccggggcctgcctttggtgcacaccctcatcacagtgtcaaaaattctgcaccataaaatgcttcattctgtcctgcaggcacccatgagcactttgaacacattgaaggctggcggcatcctcaacagattttctaaagatattgctatcctggatgatctcctccccctgacaatctttgactttatccagcttctgctgatcgtgattggagccatagcagtggttgctgtcctgcagccctacatttttgtggccaccgtgcccgtgattgttgcctttattatgctcagagcttacttcctgcaaacttctcaacagctcaaacagctagaatctgagggccggagccccatttttacccacctggtgacttccctgaagggactgtggactctgagagcattcgggcgacagccttactttgagacactgttccacaaggccctgaacttgcacactgccaactggtttctttacctgagcacactccgctggttccagatgcggatagagatgatcttcgtcatcttttttatagctgtaaccttcatttctatccttacaacaggagaaggagagggcagggtgggaatcatcctcacgctggctatgaacataatgtccaccttgcagtgggccgtgaattccagtatagatgtggattctctaatgaggagtgtctcccgggtgtttaaattcattgatatgcctactgaggggaaacccaccaagtcaacaaaaccttataagaatggacagctgagcaaggtgatgataattgagaacagccacgtgaagaaggatgacatttggcccagcgggggccagatgactgtgaaggacctgacggccaagtacaccgaaggtggaaatgccattttggaaaacatcagcttctcaatctctcctgggcagagagttggattgctgggtcgcacgggcagcggcaaatcaaccctgctcagtgccttccttcggctcctgaatacagaaggcgaaatccaaattgacggggtgagctgggacagcatcaccctgcagcagtggagaaaagcatttggggtcattccacagaaagttttcatcttctctggcactttcagaaagaacctggacccctatgagcagtggagcgaccaggagatctggaaggttgcagatgaagttggcctgcggagtgtgatagaacaatttcctggcaagctggattttgtgctggtagatggaggctgcgtgctgtcccacggccacaaacagctgatgtgcctcgcccgctccgttctttcaaaggccaaaatcttgcttttggatgagcccagtgctcacctcgacccagtgacctatcagataatccgcaggaccttaaagcaagcttttgccgactgcaccgtcatactgtgtgagcaccggattgaagcaatgctggaatgccagcagtttctggtgatcgaggagaataaggtccggcagtacgacagcatccagaagttgttgaatgagcgcagccttttccgccaggccatctccccatctgacagagtcaagctgtttccacataggaactcctctaagtgcaagtccaagccccagatcgctgccctcaaggaggaaactgaggaagaggtgcaggatacccgcctgtga

SEQ ID NO: 18 - DNA, 4443 bp, Artificial Sequence
  Artificially synthesized oligonucleotide
atgcagagaagccccctggagaaggcctctgtggtgagcaagctgttcttcagctggaccagacccatcctgagaaagggctacagacagagactggagctgtctgacatctaccagatcccctctgtggactctgccgacaacctgtctgagaagctggagagagagtgggacagagagctggccagcaagaagaaccccaagctgatcaatgccctgagaagatgcttcttctggagattcatgttctatggcatcttcctgtacctgggagaggtgaccaaggccgtgcagcccctgctgctgggcaggatcattgccagctatgaccctgacaacaaggaggagagaagcattgccatctacctgggcattggcctgtgcctgctgttcattgtgagaaccctgctgctgcaccctgccatctttggcctgcaccacattggcatgcagatgagaattgccatgttcagcctgatctacaagaagaccctgaagctgagcagcagagtgctggacaagatcagcattggccagctggtgagcctgctgagcaacaacctgaacaagtttgatgagggcctggccctggcccactttgtgtggattgcccccctgcaggtggccctgctgatgggcctgatctgggagctgctgcaggcctctgccttctgtggcctgggcttcctgattgtgctggccctgttccaggccggcctgggcagaatgatgatgaagtacagagaccagagagccggcaagatctctgagagactggtgatcacctctgagatgattgagaacatccagtctgtgaaggcctactgctgggaggaggccatggagaagatgattgagaacctgagacagacagagctgaagctgaccaggaaggccgcctatgtgagatacttcaacagctctgccttcttcttctctggcttctttgtggtgttcctgtctgtgctgccctatgccctgatcaagggcatcatcctgaggaagatcttcaccaccatcagcttctgcattgtgctgaggatggccgtgaccaggcagttcccctgggccgtgcagacctggtatgacagcctgggggccatcaacaagatccaggacttcctgcagaagcaggagtacaagaccctggagtacaacctgaccaccacagaggtggtgatggagaatgtgacagccttctgggaggagggctttggagagctgtttgagaaggccaagcagaacaacaacaacagaaagaccagcaatggagatgacagcctgttcttcagcaacttcagcctgctgggcacccctgtgctgaaggacatcaacttcaagattgagaggggccagctgctggccgtggccggcagcacaggagccggcaagaccagcctgctgatggtgatcatgggagagctggagccctctgagggcaagatcaagcactctggcagaatcagcttctgcagccagttcagctggatcatgcctggcaccatcaaggagaacatcatctttggggtgagctatgatgagtacaggtacagatctgtgatcaaggcctgccagctggaggaggacatctccaagtttgccgagaaggacaacattgtgctgggggagggaggcatcaccctgtctgggggccagagagccagaatcagcctggccagagccgtgtacaaggatgccgacctgtacctgctggacagcccctttggctacctggatgtgctgacagagaaggagatctttgagagctgtgtgtgcaagctgatggccaacaagaccaggatcctggtgaccagcaagatggagcacctgaagaaggccgacaagatcctgatcctgcatgagggcagcagctacttctatggcaccttctctgagctgcagaacctgcagcctgacttcagcagcaagctgatgggctgtgacagctttgaccagttctctgctgagagaagaaacagcatcctgacagagaccctgcacaggttcagcctggagggggatgcccctgtgagctggacagagaccaagaagcagagcttcaagcagacaggagagtttggggagaagaggaagaacagcatcctgaaccccatcaacagcatcaggaagttcagcattgtgcagaagacccccctgcagatgaatggcattgaggaggactctgatgagcccctggagagaagactgagcctggtgccagactctgagcagggagaggccatcctgcccaggatctctgtgatcagcacaggccccaccctgcaggccagaagaagacagtctgtgctgaacctgatgacccactctgtgaaccagggccagaatatccacagaaagaccacagccagcaccagaaaggtgagcctggccccccaggccaacctgacagagctggacatctacagcagaaggctgagccaggagacaggcctggagatctctgaggagatcaatgaggaggacctgaaggagtgcttctttgatgacatggagagcatccctgccgtgaccacctggaacacctacctgagatacatcacagtgcacaagagcctgatctttgtgctgatctggtgcctggtgatcttcctggccgaggtggccgccagcctggtggtgctgtggctgctgggcaacacccccctgcaggacaagggcaacagcacccacagcagaaacaacagctatgctgtgatcatcaccagcaccagcagctactatgtgttctacatctatgtgggagtggctgacaccctgctggccatgggcttcttcagaggcctgcccctggtgcacaccctgatcacagtgagcaagatcctgcaccacaagatgctgcactctgtgctgcaggcccccatgagcaccctgaacaccctgaaggctggaggcatcctgaacagattcagcaaggacattgccatcctggatgacctgctgcccctgaccatctttgacttcatccagctgctgctgattgtgattggagccattgccgtggtggccgtgctgcagccctacatctttgtggccacagtgcctgtgattgtggccttcatcatgctgagggcctacttcctgcagaccagccagcagctgaagcagctggagtctgagggcagaagccccatcttcacccacctggtgaccagcctgaagggcctgtggaccctgagggcctttggcagacagccctactttgagaccctgttccacaaggccctgaacctgcacacagccaactggttcctgtacctgagcaccctgagatggttccagatgaggattgagatgatctttgtgatcttcttcattgccgtgaccttcatcagcatcctgaccacaggggagggcgagggcagagtgggcatcatcctgaccctggccatgaacatcatgagcaccctgcagtgggccgtgaacagcagcattgatgtggacagcctgatgagatctgtgagcagagtgttcaagttcattgacatgcccacagagggcaagcccaccaagagcaccaagccctacaagaatggccagctgagcaaggtgatgatcattgagaacagccatgtgaagaaggatgacatctggccctctggaggccagatgacagtgaaggacctgacagccaagtacacagaggggggcaatgccatcctggagaacatcagcttcagcatcagccctggccagagggtgggcctgctgggcagaacaggctctggcaagagcaccctgctgtctgccttcctgaggctgctgaacacagagggagagatccagattgatggggtgagctgggacagcatcaccctgcagcagtggaggaaggcctttggggtgatcccccagaaggtgttcatcttctctggcaccttcaggaagaacctggacccctatgagcagtggtctgaccaggagatctggaaggtggccgatgaggtgggcctgagatctgtgattgagcagttccctggcaagctggactttgtgctggtggatggaggctgtgtgctgagccatggccacaagcagctgatgtgcctggccagatctgtgctgagcaaggccaagatcctgctgctggatgagccctctgcccacctggaccctgtgacctaccagatcatcagaagaaccctgaagcaggcctttgccgactgcacagtgatcctgtgtgagcacagaattgaggccatgctggagtgccagcagttcctggtgattgaggagaacaaggtgaggcagtatgacagcatccagaagctgctgaatgagagaagcctgttcagacaggccatcagcccctctgacagagtgaagctgttcccccacaggaacagcagcaagtgcaagagcaagccccagattgccgccctgaaggaggagacagaggaggaggtgcaggacaccagactgtga

SEQ ID NO: 19 - DNA, 4443 bp, Artificial Sequence
  Chemically synthesized oligonucleotide
atgcagaggagccccctggagaaggccagcgtggtgagcaagctgttcttcagctggaccaggcccatcctgaggaagggctacaggcagaggctggagctgagcgacatctaccagatccccagcgtggacagcgccgacaacctgagcgagaagctggagagggagtgggacagggagctggccagcaagaagaaccccaagctgatcaacgccctgaggaggtgcttcttctggaggttcatgttctacggcatcttcctgtacctgggcgaggtgaccaaggccgtgcagcccctgctgctgggcaggatcatcgccagctacgaccccgacaacaaggaggagaggagcatcgccatctacctgggcatcggcctgtgcctgctgttcatcgtgaggaccctgctgctgcaccccgccatcttcggcctgcaccacatcggcatgcagatgaggatcgccatgttcagcctgatctacaagaagaccctgaagctgagcagcagggtgctggacaagatcagcatcggccagctggtgagcctgctgagcaacaacctgaacaagttcgacgagggcctggccctggcccacttcgtgtggatcgcccccctgcaggtggccctgctgatgggcctgatctgggagctgctgcaggccagcgccttctgcggcctgggcttcctgatcgtgctggccctgttccaggccggcctgggcaggatgatgatgaagtacagggaccagagggccggcaagatcagcgagaggctggtgatcaccagcgagatgatcgagaacatccagagcgtgaaggcctactgctgggaggaggccatggagaagatgatcgagaacctgaggcagaccgagctgaagctgaccaggaaggccgcctacgtgaggtacttcaacagcagcgccttcttcttcagcggcttcttcgtggtgttcctgagcgtgctgccctacgccctgatcaagggcatcatcctgaggaagatcttcaccaccatcagcttctgcatcgtgctgaggatggccgtgaccaggcagttcccctgggccgtgcagacctggtacgacagcctgggcgccatcaacaagatccaggacttcctgcagaagcaggagtacaagaccctggagtacaacctgaccaccaccgaggtggtgatggagaacgtgaccgccttctgggaggagggcttcggcgagctgttcgagaaggccaagcagaacaacaacaacaggaagaccagcaacggcgacgacagcctgttcttcagcaacttcagcctgctgggcacccccgtgctgaaggacatcaacttcaagatcgagaggggccagctgctggccgtggccggcagcaccggcgccggcaagaccagcctgctgatggtgatcatgggcgagctggagcccagcgagggcaagatcaagcacagcggcaggatcagcttctgcagccagttcagctggatcatgcccggcaccatcaaggagaacatcatcttcggcgtgagctacgacgagtacaggtacaggagcgtgatcaaggcctgccagctggaggaggacatcagcaagttcgccgagaaggacaacatcgtgctgggcgagggcggcatcaccctgagcggcggccagagggccaggatcagcctggccagggccgtgtacaaggacgccgacctgtacctgctggacagccccttcggctacctggacgtgctgaccgagaaggagatcttcgagagctgcgtgtgcaagctgatggccaacaagaccaggatcctggtgaccagcaagatggagcacctgaagaaggccgacaagatcctgatcctgcacgagggcagcagctacttctacggcaccttcagcgagctgcagaacctgcagcccgacttcagcagcaagctgatgggctgcgacagcttcgaccagttcagcgccgagaggaggaacagcatcctgaccgagaccctgcacaggttcagcctggagggcgacgcccccgtgagctggaccgagaccaagaagcagagcttcaagcagaccggcgagttcggcgagaagaggaagaacagcatcctgaaccccatcaacagcatcaggaagttcagcatcgtgcagaagacccccctgcagatgaacggcatcgaggaggacagcgacgagcccctggagaggaggctgagcctggtgcccgacagcgagcagggcgaggccatcctgcccaggatcagcgtgatcagcaccggccccaccctgcaggccaggaggaggcagagcgtgctgaacctgatgacccacagcgtgaaccagggccagaacatccacaggaagaccaccgccagcaccaggaaggtgagcctggccccccaggccaacctgaccgagctggacatctacagcaggaggctgagccaggagaccggcctggagatcagcgaggagatcaacgaggaggacctgaaggagtgcttcttcgacgacatggagagcatccccgccgtgaccacctggaacacctacctgaggtacatcaccgtgcacaagagcctgatcttcgtgctgatctggtgcctggtgatcttcctggccgaggtggccgccagcctggtggtgctgtggctgctgggcaacacccccctgcaggacaagggcaacagcacccacagcaggaacaacagctacgccgtgatcatcaccagcaccagcagctactacgtgttctacatctacgtgggcgtggccgacaccctgctggccatgggcttcttcaggggcctgcccctggtgcacaccctgatcaccgtgagcaagatcctgcaccacaagatgctgcacagcgtgctgcaggcccccatgagcaccctgaacaccctgaaggccggcggcatcctgaacaggttcagcaaggacatcgccatcctggacgacctgctgcccctgaccatcttcgacttcatccagctgctgctgatcgtgatcggcgccatcgccgtggtggccgtgctgcagccctacatcttcgtggccaccgtgcccgtgatcgtggccttcatcatgctgagggcctacttcctgcagaccagccagcagctgaagcagctggagagcgagggcaggagccccatcttcacccacctggtgaccagcctgaagggcctgtggaccctgagggccttcggcaggcagccctacttcgagaccctgttccacaaggccctgaacctgcacaccgccaactggttcctgtacctgagcaccctgaggtggttccagatgaggatcgagatgatcttcgtgatcttcttcatcgccgtgaccttcatcagcatcctgaccaccggcgagggcgagggcagggtgggcatcatcctgaccctggccatgaacatcatgagcaccctgcagtgggccgtgaacagcagcatcgacgtggacagcctgatgaggagcgtgagcagggtgttcaagttcatcgacatgcccaccgagggcaagcccaccaagagcaccaagccctacaagaacggccagctgagcaaggtgatgatcatcgagaacagccacgtgaagaaggacgacatctggcccagcggcggccagatgaccgtgaaggacctgaccgccaagtacaccgagggcggcaacgccatcctggagaacatcagcttcagcatcagccccggccagagggtgggcctgctgggcaggaccggcagcggcaagagcaccctgctgagcgccttcctgaggctgctgaacaccgagggcgagatccagatcgacggcgtgagctgggacagcatcaccctgcagcagtggaggaaggccttcggcgtgatcccccagaaggtgttcatcttcagcggcaccttcaggaagaacctggacccctacgagcagtggagcgaccaggagatctggaaggtggccgacgaggtgggcctgaggagcgtgatcgagcagttccccggcaagctggacttcgtgctggtggacggcggctgcgtgctgagccacggccacaagcagctgatgtgcctggccaggagcgtgctgagcaaggccaagatcctgctgctggacgagcccagcgcccacctggaccccgtgacctaccagatcatcaggaggaccctgaagcaggccttcgccgactgcaccgtgatcctgtgcgagcacaggatcgaggccatgctggagtgccagcagttcctggtgatcgaggagaacaaggtgaggcagtacgacagcatccagaagctgctgaacgagaggagcctgttcaggcaggccatcagccccagcgacagggtgaagctgttcccccacaggaacagcagcaagtgcaagagcaagccccagatcgccgccctgaaggaggagaccgaggaggaggtgcaggacaccaggctgtga

SEQ ID NO: 20 - DNA, 4443 bp, Artificial Sequence
  Chemically synthesized oligonucleotide
atgcagagatcccctctggagaaggcctcagtggtgtccaagcttttcttctcctggaccaggcccattttaagaaagggctacaggcagagacttgagctgtctgacatctatcagatcccttctgtggattctgctgacaatcttagtgaaaaattggaaagggagtgggacagagagctggcaagtaaaaagaaccccaagctgattaatgccctgaggcgctgctttttttggagattcatgttctatggcatattcctctaccttggagaagtaaccaaagctgtacagcctctcctccttggcagaatcattgcctcctatgatcctgataacaaggaggagagaagcatagccatctacctgggcattgggctgtgcctcttgtttattgtgaggacccttctcttgcaccctgccatctttggccttcatcacattggcatgcaaatgagaatagcaatgtttagtcttatttacaaaaaaacattaaaactctcttccagggtgttggacaagatcagtattggacaactggtcagcctgctgagcaacaacctgaacaagtttgatgaaggactggccctggcccactttgtctggattgccccccttcaggtggctcttttgatgggcctgatctgggaactcctgcaggcctctgccttctgtgggttaggcttcctgatagtgctagctctctttcaggcagggttgggtagaatgatgatgaagtacagagaccagagggctgggaagatatctgagaggctggtcattacttctgaaatgatagaaaacatccagtctgttaaagcttactgctgggaggaggctatggaaaagatgattgagaacttgaggcaaacagagctcaagctgactaggaaggcagcctatgtcaggtatttcaacagcagtgctttcttcttctcaggctttttcgtggtcttcttgagtgttctgccctatgccctcatcaaggggataattttgagaaagattttcaccactatttccttttgcattgtcctgaggatggctgtcaccaggcaattcccctgggctgtgcagacatggtatgactctctgggggccatcaacaaaatccaagatttcctgcagaagcaggagtacaagaccctggaatacaacctcaccaccacagaagttgtgatggagaatgtgactgcattctgggaggaaggatttggggagctgtttgagaaagcaaaacaaaacaataataacaggaaaaccagcaatggagatgactccctgttcttttccaacttctctttgttgggcacccctgtcctgaaagatataaactttaaaattgaaagagggcagctgttggcagttgctggctccacaggagctggaaaaacttcactactgatggtgatcatgggggagttagaaccctctgaagggaaaataaaacattctgggaggattagtttctgcagccagttcagctggatcatgcctgggaccattaaagaaaatattatatttggagtgagctatgatgaatatagatataggagtgtcatcaaagcctgtcagttggaggaagacatcagcaaatttgcagagaaagacaacattgttctgggtgaaggtggcatcaccctgtcaggagggcaaagggccaggatcagcttggccagagcagtctataaagatgctgatctgtacctcctggatagcccttttggctatctggatgttttgacagagaaggaaatttttgagtcctgtgtctgcaagttaatggcaaataaaacaaggatacttgtgacctcaaaaatggaacacctgaagaaggctgacaaaattctgatcctgcatgagggcagcagctacttttatggaacattttctgaactgcagaatttgcaaccagacttttcatcaaagctcatgggatgtgacagttttgatcagttttctgcagaaaggagaaactccattttgactgagaccctgcacaggttcagtctggagggggatgccccagtgagttggactgagacaaagaaacagagcttcaagcagactggagagtttggagaaaagaggaaaaactcaattctcaatcccatcaatagcatcaggaagttcagcatagttcagaagactcctttgcagatgaatgggattgaagaggactcagatgagcccctggaaaggagactctccttggtgccagattcagagcagggggaagccatactgccaaggatctctgtgatttctacagggcccaccctccaagcaagaaggagacagtcagttttaaacctgatgacccactctgtcaaccagggacagaacattcatagaaagacaacagcatctacaagaaaagtttcactggcccctcaagccaatttaactgaactagatatctacagcaggaggctcagccaagaaacaggcctggagatctcagaagaaataaatgaggaggatttgaaggaatgcttctttgatgatatggagagcatcccagctgtcacaacctggaacacctacctgagatacatcacagtgcacaaatccctcatctttgtacttatatggtgccttgtcatcttcttagctgaggtggctgcttccctggtggtgctgtggctgctgggaaacacacccctccaggataaagggaactctactcacagcaggaacaacagttatgctgtgatcatcaccagtacctcctcctactatgtgttctacatttatgttggagttgcagacacattgcttgccatgggtttttttagaggactccccctggtgcatactctcatcactgtttccaaaatccttcaccacaagatgctgcacagtgtactacaggctcccatgagcaccctcaacactcttaaagcaggaggaatcttgaacagatttagcaaggacattgcaattcttgatgacctgcttccactgaccatctttgacttcatccagcttctgctcattgtaattggtgccattgctgtggtagcagtgctccagccatatatttttgtggccactgtgcctgttattgtggccttcattatgttgagagcctacttcctgcagacctctcagcagctcaagcaacttgaaagtgagggcaggagccccatatttacacacttggtcacttccctcaaaggcctctggacactcagagcttttggaagacaaccttattttgaaactctcttccacaaggctctgaatctccacacagccaactggtttctgtatctttcaacactgcgctggttccagatgaggattgagatgatctttgttatcttcttcatagctgttaccttcatctctattctgacaactggtgagggggaagggagagtaggcatcatcctcacactagccatgaacataatgtctaccttacaatgggccgtgaacagctccatagatgtggacagcctcatgagaagtgtgtcaagagttttcaaattcattgacatgcccacagaaggcaaaccaaccaagagcacaaaaccctacaagaatggccagctgagtaaggtcatgatcattgaaaattctcatgtgaagaaggatgatatttggcccagtgggggccagatgacagtcaaggacctcactgccaaatacacagagggtggaaatgctatcctagagaacatctccttctccatctccccaggccaaagagttggcttgctgggcaggactggcagtggcaagtccaccttgctctcagcatttctcaggcttttaaatacagagggagagattcaaattgatggggtgtcttgggatagtataacacttcaacagtggaggaaagcctttggtgtgattcctcagaaagtgtttatcttctctggcactttcagaaaaaatctggacccctatgaacagtggagtgaccaggaaatctggaaggtggcagatgaagtgggcctaagatcagtcatagagcagtttcctggaaagttggattttgtgcttgtagatggaggctgtgtgctgtcccatggccataaacagctaatgtgcctggctaggtcagtgctgagcaaggccaagatcctgctgttagatgagccttcagcccatctggaccctgtgacataccagattatcagaagaactctgaagcaggcctttgctgactgcactgtcatcctgtgtgagcacagaattgaggccatgctggagtgccagcagttccttgttatagaagagaataaggttaggcagtatgacagcattcagaaactgctaaatgaaagatctctcttcaggcaagctatttcaccatctgatagagtgaaactttttccccacagaaattcctctaaatgtaaatctaagccccagatagctgccttgaaagaggagactgaagaagaagtccaggacaccagactgtga

SEQ ID NO: 21 - DNA, 4443 bp, Artificial Sequence
  Chemically synthesized oligonucleotide
atgcagagatccccgctggagaaggcatctgtggtgtcaaaactgttctttagctggacaaggcccatccttaggaaagggtacagacagaggttggagctgtcagacatatatcagatcccttcagtggactctgcagacaacctctctgaaaagctggagagggaatgggacagggaactggccagcaaaaaaaaccctaaactgattaatgccctgaggaggtgcttcttttggagattcatgttctatgggatcttcctttacctgggggaggtgactaaagctgttcagcctcttcttctggggaggattattgcctcctatgacccagacaacaaagaagaaagaagcatagccatttacttaggcataggcctctgcttgctcttcatagttagaaccctcctactccacccagccatctttggtctccaccacataggtatgcagatgagaatagcaatgttctccttgatctacaagaagaccctcaagctgtccagcagggtgctggacaagatctccataggccagttagtcagtctactgtccaataacttaaataagtttgatgagggactggcactggcacattttgtgtggattgcccccctccaagtggcccttcttatgggccttatctgggagctgttgcaggcctctgctttctgtggcctgggtttcctcatagtcctagccttattccaggctggactgggcagaatgatgatgaagtatagggaccaaagagcagggaagatttctgaaaggctggttataacttctgagatgattgagaacattcagtcagtgaaagcttactgctgggaagaagctatggaaaaaatgattgaaaatctcagacagactgaattaaagttgaccaggaaagctgcttatgtcagatacttcaactcctcagccttctttttttctggcttctttgttgtattcctttcagtcctcccctatgccctgattaagggcattatcttgaggaaaattttcacaaccatctccttttgtattgtcctcaggatggctgttacaaggcaatttccttgggctgtgcaaacttggtatgatagccttggagcaatcaacaagatccaggatttcctgcaaaagcaggagtacaagacattggaatacaaccttaccaccactgaggtggtgatggaaaatgtgactgccttctgggaggaggggtttggagagctgtttgagaaagccaaacagaacaacaacaatagaaagacctctaatggtgatgattccctgttcttttctaactttagtcttctggggaccccagttctgaaagatattaactttaaaattgaaaggggacagttgctggctgtggctgggtccactggggctgggaagacaagcctgctcatggtgatcatgggagagctggaacccagtgaaggaaagatcaaacactcaggcaggatctccttctgcagccagttctcatggattatgccaggcactattaaagaaaatatcatctttggtgtaagctatgatgagtacaggtatagatctgtaattaaagcctgccagctggaggaagacatctctaagtttgctgagaaggataacattgtgttgggggaagggggcatcaccctttctggtgggcagagggctaggatctcccttgctagggcagtatacaaggatgctgacttgtacctcttggatagtccttttggctacctagatgtgctgacagagaaagaaatatttgaaagctgtgtgtgtaagctcatggctaacaagaccaggatcctggtcaccagtaaaatggaacacctcaaaaaagcagacaagatccttattctccatgagggctcctcctacttctatgggaccttcagtgagctgcagaatctgcagccagacttctcctcaaaacttatgggctgtgactcctttgaccaattctctgcagaaagaaggaatagcatactgacagaaacactgcatagattctccctggaaggagatgccccagtgagttggacagaaaccaaaaagcagagcttcaagcagactggtgagtttggtgaaaagaggaagaattctatcctgaaccccatcaatagcatcaggaaatttagcatagtccaaaagacccccctccagatgaatggaatagaggaggatagtgatgagcctcttgagagaaggctgtccctggttccagacagtgaacagggtgaagccattcttccgaggatcagtgtcatctccactgggcccacattgcaggccagaagaagacagtctgttctgaatttgatgacacattctgtgaatcaaggccagaatatccatagaaaaaccactgccagcaccagaaaagtttctctagccccccaggctaacctgactgagttagacatctacagcagaaggctgagccaagagactggcttggaaatatctgaggagatcaatgaggaggacctcaaggagtgcttctttgatgacatggagtcaatccctgcagtcactacatggaacacttacctaaggtacatcacagttcataagagcctcatctttgtcctcatatggtgtctggtcatctttttagcagaagtggctgccagcctagttgtgctgtggttactgggcaatacacctcttcaggacaaaggcaatagcacacacagcagaaacaactcctatgcagtgatcatcacctctacaagctcttactatgtattctatatatatgtgggagtggcagatactctcctggccatgggattcttcaggggattacctctagttcacacattgatcacagtgtcaaaaattctccaccacaagatgttacacagtgtcctgcaagccccaatgtctactctgaacacacttaaggcaggtggaattttgaataggtttagcaaggacatagctatcctggatgatctcctccctctgaccatctttgacttcatccagttactgctcattgtaattggagccattgcagtggtagcagtcctacagccttacatttttgtggctactgttcctgttattgtggccttcattatgctaagagcttacttcctgcaaacaagccaacagttgaaacagctagaaagtgagggaaggtcccccatcttcacccacctggtgacatcactcaaggggctatggactcttagggcttttgggagacagccgtactttgagaccttattccataaggcccttaacctccatacagcaaactggttcttatacctgagtactctgaggtggtttcaaatgaggattgaaatgatttttgtgatcttcttcattgctgtgaccttcatctcaatcttgaccacaggagagggggagggcagggtgggcatcatactgaccttggccatgaacattatgtcaaccctgcagtgggctgtcaatagctccattgatgtggacagtctgatgaggagtgtctccagggtcttcaagtttattgacatgccaactgagggcaaacccaccaaaagcactaagccatataaaaatggccaactgtccaaagtgatgatcattgaaaattcacatgtaaagaaggatgatatctggccctctggaggacagatgacagtgaaagacctgactgccaagtacacagagggtggtaatgccattcttgagaacattagtttcagtatttccccggggcaaagggtgggcctccttggcagaacaggctctggcaagagtaccctgctgtcagcctttttaagactgttgaacactgagggagaaattcagattgatggtgtctcctgggatagcatcaccctccagcagtggagaaaagcttttggagtgatcccgcaaaaggttttcatcttttcaggcaccttccggaagaacctggacccctatgagcagtggtctgaccaggaaatatggaaggtagctgatgaagttgggcttaggtcagtcatagagcagttcccaggcaaactggactttgtcctggtggatggtggatgtgtactgagtcatgggcacaaacagctgatgtgcctagccaggtctgtgctcagcaaggcaaagatattgctgcttgatgaacccagtgcccatctggacccagtcacatatcagatcatcagaagaacattgaagcaggcctttgctgattgcacagttatcctctgtgagcacaggattgaggccatgctggagtgccagcagtttctggtgattgaggagaataaagtaaggcagtatgactccatccagaagctgctcaatgaaagaagcctctttagacaagctatctccccctcagacagggtcaaattgttccctcacagaaacagcagcaagtgcaagagcaagccccaaattgcagccttgaaagaggagacagaggaagaggtgcaggacaccagactctga

SEQ ID NO: 22 - DNA, 4443 bp, Artificial Sequence
  Chemically synthesized oligonucleotide
atgcagagaagccccctggagaaggccagcgtggtgagcaagctgttcttcagctggaccagacccatcctgagaaagggctacagacagagactggagctgagcgacatctaccagatccccagcgtggacagcgccgacaacctgagcgagaagctggagagagagtgggacagagagctggccagcaagaagaaccccaagctgatcaacgccctgagaagatgcttcttctggagattcatgttctacggcatcttcctgtacctgggcgaggtgaccaaggccgtgcagcccctgctgctgggcagaatcatcgccagctacgaccccgacaacaaggaggagagaagcatcgccatctacctgggcatcggcctgtgcctgctgttcatcgtgagaaccctgctgctgcaccccgccatcttcggcctgcaccacatcggcatgcagatgagaatcgccatgttcagcctgatctacaagaagaccctgaagctgagcagcagagtgctggacaagatcagcatcggccagctggtgagcctgctgagcaacaacctgaacaagttcgacgagggcctggccctggcccacttcgtgtggatcgcccccctgcaggtggccctgctgatgggcctgatctgggagctgctgcaggccagcgccttctgcggcctgggcttcctgatcgtgctggccctgttccaggccggcctgggcagaatgatgatgaagtacagagaccagagagccggcaagatcagcgagagactggtgatcaccagcgagatgatcgagaacatccagagcgtgaaggcctactgctgggaggaggccatggagaagatgatcgagaacctgagacagaccgagctgaagctgaccagaaaggccgcctacgtgagatacttcaacagcagcgccttcttcttcagcggcttcttcgtggtgttcctgagcgtgctgccctacgccctgatcaagggcatcatcctgagaaagatcttcaccaccatcagcttctgcatcgtgctgagaatggccgtgaccagacagttcccctgggccgtgcagacctggtacgacagcctgggcgccatcaacaagatccaggacttcctgcagaagcaggagtacaagaccctggagtacaacctgaccaccaccgaggtggtgatggagaacgtgaccgccttctgggaggagggcttcggcgagctgttcgagaaggccaagcagaacaacaacaacagaaagaccagcaacggcgacgacagcctgttcttcagcaacttcagcctgctgggcacccccgtgctgaaggacatcaacttcaagatcgagagaggccagctgctggccgtggccggcagcaccggcgccggcaagaccagcctgctgatggtgatcatgggcgagctggagcccagcgagggcaagatcaagcacagcggcagaatcagcttctgcagccagttcagctggatcatgcccggcaccatcaaggagaacatcatcttcggcgtgagctacgacgagtacagatacagaagcgtgatcaaggcctgccagctggaggaggacatcagcaagttcgccgagaaggacaacatcgtgctgggcgagggcggcatcaccctgagcggcggccagagagccagaatcagcctggccagagccgtgtacaaggacgccgacctgtacctgctggacagccccttcggctacctggacgtgctgaccgagaaggagatcttcgagagctgcgtgtgcaagctgatggccaacaagaccagaatcctggtgaccagcaagatggagcacctgaagaaggccgacaagatcctgatcctgcacgagggcagcagctacttctacggcaccttcagcgagctgcagaacctgcagcccgacttcagcagcaagctgatgggctgcgacagcttcgaccagttcagcgccgagagaagaaacagcatcctgaccgagaccctgcacagattcagcctggagggcgacgcccccgtgagctggaccgagaccaagaagcagagcttcaagcagaccggcgagttcggcgagaagagaaagaacagcatcctgaaccccatcaacagcatcagaaagttcagcatcgtgcagaagacccccctgcagatgaacggcatcgaggaggacagcgacgagcccctggagagaagactgagcctggtgcccgacagcgagcagggcgaggccatcctgcccagaatcagcgtgatcagcaccggccccaccctgcaggccagaagaagacagagcgtgctgaacctgatgacccacagcgtgaaccagggccagaacatccacagaaagaccaccgccagcaccagaaaggtgagcctggccccccaggccaacctgaccgagctggacatctacagcagaagactgagccaggagaccggcctggagatcagcgaggagatcaacgaggaggacctgaaggagtgcttcttcgacgacatggagagcatccccgccgtgaccacctggaacacctacctgagatacatcaccgtgcacaagagcctgatcttcgtgctgatctggtgcctggtgatcttcctggccgaggtggccgccagcctggtggtgctgtggctgctgggcaacacccccctgcaggacaagggcaacagcacccacagcagaaacaacagctacgccgtgatcatcaccagcaccagcagctactacgtgttctacatctacgtgggcgtggccgacaccctgctggccatgggcttcttcagaggcctgcccctggtgcacaccctgatcaccgtgagcaagatcctgcaccacaagatgctgcacagcgtgctgcaggcccccatgagcaccctgaacaccctgaaggccggcggcatcctgaacagattcagcaaggacatcgccatcctggacgacctgctgcccctgaccatcttcgacttcatccagctgctgctgatcgtgatcggcgccatcgccgtggtggccgtgctgcagccctacatcttcgtggccaccgtgcccgtgatcgtggccttcatcatgctgagagcctacttcctgcagaccagccagcagctgaagcagctggagagcgagggcagaagccccatcttcacccacctggtgaccagcctgaagggcctgtggaccctgagagccttcggcagacagccctacttcgagaccctgttccacaaggccctgaacctgcacaccgccaactggttcctgtacctgagcaccctgagatggttccagatgagaatcgagatgatcttcgtgatcttcttcatcgccgtgaccttcatcagcatcctgaccaccggcgagggcgagggcagagtgggcatcatcctgaccctggccatgaacatcatgagcaccctgcagtgggccgtgaacagcagcatcgacgtggacagcctgatgagaagcgtgagcagagtgttcaagttcatcgacatgcccaccgagggcaagcccaccaagagcaccaagccctacaagaacggccagctgagcaaggtgatgatcatcgagaacagccacgtgaagaaggacgacatctggcccagcggcggccagatgaccgtgaaggacctgaccgccaagtacaccgagggcggcaacgccatcctggagaacatcagcttcagcatcagccccggccagagagtgggcctgctgggcagaaccggcagcggcaagagcaccctgctgagcgccttcctgagactgctgaacaccgagggcgagatccagatcgacggcgtgagctgggacagcatcaccctgcagcagtggagaaaggccttcggcgtgatcccccagaaggtgttcatcttcagcggcaccttcagaaagaacctggacccctacgagcagtggagcgaccaggagatctggaaggtggccgacgaggtgggcctgagaagcgtgatcgagcagttccccggcaagctggacttcgtgctggtggacggcggctgcgtgctgagccacggccacaagcagctgatgtgcctggccagaagcgtgctgagcaaggccaagatcctgctgctggacgagcccagcgcccacctggaccccgtgacctaccagatcatcagaagaaccctgaagcaggccttcgccgactgcaccgtgatcctgtgcgagcacagaatcgaggccatgctggagtgccagcagttcctggtgatcgaggagaacaaggtgagacagtacgacagcatccagaagctgctgaacgagagaagcctgttcagacaggccatcagccccagcgacagagtgaagctgttcccccacagaaacagcagcaagtgcaagagcaagccccagatcgccgccctgaaggaggagaccgaggaggaggtgcaggacaccagactgtga

SEQ ID NO: 23 - DNA, 4443 bp, Artificial Sequence
  Chemically synthesized oligonucleotide
atgcagcgcagccccctggagaaggccagcgtggtgagcaagctgttcttcagctggacccgccccatcctgcgcaagggctaccgccagcgcctggagctgagcgacatctaccagatccccagcgtggacagcgccgacaacctgagcgagaagctggagcgcgagtgggaccgcgagctggccagcaagaagaaccccaagctgatcaacgccctgcgccgctgcttcttctggcgcttcatgttctacggcatcttcctgtacctgggcgaggtgaccaaggccgtgcagcccctgctgctgggccgcatcatcgccagctacgaccccgacaacaaggaggagcgcagcatcgccatctacctgggcatcggcctgtgcctgctgttcatcgtgcgcaccctgctgctgcaccccgccatcttcggcctgcaccacatcggcatgcagatgcgcatcgccatgttcagcctgatctacaagaagaccctgaagctgagcagccgcgtgctggacaagatcagcatcggccagctggtgagcctgctgagcaacaacctgaacaagttcgacgagggcctggccctggcccacttcgtgtggatcgcccccctgcaggtggccctgctgatgggcctgatctgggagctgctgcaggccagcgccttctgcggcctgggcttcctgatcgtgctggccctgttccaggccggcctgggccgcatgatgatgaagtaccgcgaccagcgcgccggcaagatcagcgagcgcctggtgatcaccagcgagatgatcgagaacatccagagcgtgaaggcctactgctgggaggaggccatggagaagatgatcgagaacctgcgccagaccgagctgaagctgacccgcaaggccgcctacgtgcgctacttcaacagcagcgccttcttcttcagcggcttcttcgtggtgttcctgagcgtgctgccctacgccctgatcaagggcatcatcctgcgcaagatcttcaccaccatcagcttctgcatcgtgctgcgcatggccgtgacccgccagttcccctgggccgtgcagacctggtacgacagcctgggcgccatcaacaagatccaggacttcctgcagaagcaggagtacaagaccctggagtacaacctgaccaccaccgaggtggtgatggagaacgtgaccgccttctgggaggagggcttcggcgagctgttcgagaaggccaagcagaacaacaacaaccgcaagaccagcaacggcgacgacagcctgttcttcagcaacttcagcctgctgggcacccccgtgctgaaggacatcaacttcaagatcgagcgcggccagctgctggccgtggccggcagcaccggcgccggcaagaccagcctgctgatggtgatcatgggcgagctggagcccagcgagggcaagatcaagcacagcggccgcatcagcttctgcagccagttcagctggatcatgcccggcaccatcaaggagaacatcatcttcggcgtgagctacgacgagtaccgctaccgcagcgtgatcaaggcctgccagctggaggaggacatcagcaagttcgccgagaaggacaacatcgtgctgggcgagggcggcatcaccctgagcggcggccagcgcgcccgcatcagcctggcccgcgccgtgtacaaggacgccgacctgtacctgctggacagccccttcggctacctggacgtgctgaccgagaaggagatcttcgagagctgcgtgtgcaagctgatggccaacaagacccgcatcctggtgaccagcaagatggagcacctgaagaaggccgacaagatcctgatcctgcacgagggcagcagctacttctacggcaccttcagcgagctgcagaacctgcagcccgacttcagcagcaagctgatgggctgcgacagcttcgaccagttcagcgccgagcgccgcaacagcatcctgaccgagaccctgcaccgcttcagcctggagggcgacgcccccgtgagctggaccgagaccaagaagcagagcttcaagcagaccggcgagttcggcgagaagcgcaagaacagcatcctgaaccccatcaacagcatccgcaagttcagcatcgtgcagaagacccccctgcagatgaacggcatcgaggaggacagcgacgagcccctggagcgccgcctgagcctggtgcccgacagcgagcagggcgaggccatcctgccccgcatcagcgtgatcagcaccggccccaccctgcaggcccgccgccgccagagcgtgctgaacctgatgacccacagcgtgaaccagggccagaacatccaccgcaagaccaccgccagcacccgcaaggtgagcctggccccccaggccaacctgaccgagctggacatctacagccgccgcctgagccaggagaccggcctggagatcagcgaggagatcaacgaggaggacctgaaggagtgcttcttcgacgacatggagagcatccccgccgtgaccacctggaacacctacctgcgctacatcaccgtgcacaagagcctgatcttcgtgctgatctggtgcctggtgatcttcctggccgaggtggccgccagcctggtggtgctgtggctgctgggcaacacccccctgcaggacaagggcaacagcacccacagccgcaacaacagctacgccgtgatcatcaccagcaccagcagctactacgtgttctacatctacgtgggcgtggccgacaccctgctggccatgggcttcttccgcggcctgcccctggtgcacaccctgatcaccgtgagcaagatcctgcaccacaagatgctgcacagcgtgctgcaggcccccatgagcaccctgaacaccctgaaggccggcggcatcctgaaccgcttcagcaaggacatcgccatcctggacgacctgctgcccctgaccatcttcgacttcatccagctgctgctgatcgtgatcggcgccatcgccgtggtggccgtgctgcagccctacatcttcgtggccaccgtgcccgtgatcgtggccttcatcatgctgcgcgcctacttcctgcagaccagccagcagctgaagcagctggagagcgagggccgcagccccatcttcacccacctggtgaccagcctgaagggcctgtggaccctgcgcgccttcggccgccagccctacttcgagaccctgttccacaaggccctgaacctgcacaccgccaactggttcctgtacctgagcaccctgcgctggttccagatgcgcatcgagatgatcttcgtgatcttcttcatcgccgtgaccttcatcagcatcctgaccaccggcgagggcgagggccgcgtgggcatcatcctgaccctggccatgaacatcatgagcaccctgcagtgggccgtgaacagcagcatcgacgtggacagcctgatgcgcagcgtgagccgcgtgttcaagttcatcgacatgcccaccgagggcaagcccaccaagagcaccaagccctacaagaacggccagctgagcaaggtgatgatcatcgagaacagccacgtgaagaaggacgacatctggcccagcggcggccagatgaccgtgaaggacctgaccgccaagtacaccgagggcggcaacgccatcctggagaacatcagcttcagcatcagccccggccagcgcgtgggcctgctgggccgcaccggcagcggcaagagcaccctgctgagcgccttcctgcgcctgctgaacaccgagggcgagatccagatcgacggcgtgagctgggacagcatcaccctgcagcagtggcgcaaggccttcggcgtgatcccccagaaggtgttcatcttcagcggcaccttccgcaagaacctggacccctacgagcagtggagcgaccaggagatctggaaggtggccgacgaggtgggcctgcgcagcgtgatcgagcagttccccggcaagctggacttcgtgctggtggacggcggctgcgtgctgagccacggccacaagcagctgatgtgcctggcccgcagcgtgctgagcaaggccaagatcctgctgctggacgagcccagcgcccacctggaccccgtgacctaccagatcatccgccgcaccctgaagcaggccttcgccgactgcaccgtgatcctgtgcgagcaccgcatcgaggccatgctggagtgccagcagttcctggtgatcgaggagaacaaggtgcgccagtacgacagcatccagaagctgctgaacgagcgcagcctgttccgccaggccatcagccccagcgaccgcgtgaagctgttcccccaccgcaacagcagcaagtgcaagagcaagccccagatcgccgccctgaaggaggagaccgaggaggaggtgcaggacacccgcctgtaa

SEQ ID NO: 24 - DNA, 4443 bp, Artificial Sequence
  Chemically synthesized oligonucleotide
atgcagagaagccccctggagaaggccagcgtggtgagcaagctgttcttcagctggaccagacccatcctgagaaagggctacagacagagactggagctgagcgacatctaccagatccccagcgtggacagcgccgacaacctgagcgagaagctggagagagagtgggacagagagctggccagcaagaagaaccccaagctgatcaacgccctgagaagatgcttcttctggagattcatgttctacggcatcttcctgtacctgggcgaggtgaccaaggccgtgcagcccctgctgctgggcagaatcatcgccagctacgaccccgacaacaaggaggagagaagcatcgccatctacctgggcatcggcctgtgcctgctgttcatcgtgagaaccctgctgctgcaccccgccatcttcggcctgcaccacatcggcatgcagatgagaatcgccatgttcagcctgatctacaagaagaccctgaagctgagcagcagagtgctggacaagatcagcatcggccagctggtgagcctgctgagcaacaacctgaacaagttcgacgagggcctggccctggcccacttcgtgtggatcgcccccctgcaggtggccctgctgatgggcctgatctgggagctgctgcaggccagcgccttctgcggcctgggcttcctgatcgtgctggccctgttccaggccggcctgggcagaatgatgatgaagtacagggaccagagagccggcaagatcagcgagagactggtgatcaccagcgagatgatcgagaacatccagagcgtgaaggcctactgctgggaggaggccatggagaagatgatcgagaacctgagacagaccgagctgaagctgaccagaaaggccgcctacgtgagatacttcaacagcagcgccttcttcttcagcggcttcttcgtggtgttcctgagcgtgctgccctacgccctgatcaagggcatcatcctgagaaagatcttcaccaccatcagcttctgcatcgtgctgagaatggccgtgaccagacagttcccctgggccgtgcagacctggtacgacagcctgggcgccatcaacaagatccaggacttcctgcagaagcaggagtacaagaccctggagtacaacctgaccaccaccgaggtggtgatggagaacgtgaccgccttctgggaggagggcttcggcgagctgttcgagaaggccaagcagaacaacaacaacagaaagaccagcaacggcgacgacagcctgttcttcagcaacttcagcctgctgggcacccccgtgctgaaggacatcaacttcaagatcgagagaggccagctgctggccgtggccggcagcaccggcgccggcaagaccagcctgctgatggtgatcatgggcgagctggagcccagcgagggcaagatcaagcacagcggcagaatcagcttctgcagccagttcagctggatcatgcccggcaccatcaaggagaacatcatcttcggcgtgagctacgacgagtacagatacagaagcgtgatcaaggcctgccagctggaggaggacatcagcaagttcgccgagaaggacaacatcgtgctgggcgagggcggcatcaccctgagcggcggccagagagccagaatcagcctggccagagccgtgtacaaggacgccgacctgtacctgctggacagccccttcggctacctggacgtgctgaccgagaaggagatcttcgagagctgcgtgtgcaagctgatggccaacaagaccagaatcctggtgaccagcaagatggagcacctgaagaaggccgacaagatcctgatcctgcacgagggcagcagctacttctacggcaccttcagcgagctgcagaacctgcagcccgacttcagcagcaagctgatgggctgcgacagcttcgaccagttcagcgccgagagaagaaacagcatcctgaccgagaccctgcacagattcagcctggagggcgacgcccccgtgagctggaccgagaccaagaagcagagcttcaagcagaccggcgagttcggcgagaagagaaagaacagcatcctgaaccccatcaacagcatcagaaagttcagcatcgtgcagaagacccccctgcagatgaacggcatcgaggaggacagcgacgagcccctggagagaagactgagcctggtgcccgacagcgagcagggcgaggccatcctgcccagaatcagcgtgatcagcaccggccccaccctgcaggccagaagaagacagagcgtgctgaacctgatgacccacagcgtgaaccagggccagaacatccacagaaagaccaccgccagcaccagaaaggtgagcctggccccccaggccaacctgaccgagctggacatctacagcagaagactgagccaggagaccggcctggagatcagcgaggagatcaacgaggaggacctgaaggagtgcttcttcgacgacatggagagcatccccgccgtgaccacctggaacacctacctgagatacatcaccgtgcacaagagcctgatcttcgtgctgatctggtgcctggtgatcttcctggccgaggtggccgccagcctggtggtgctgtggctgctgggcaacacccccctgcaggacaagggcaacagcacccacagcagaaacaacagctacgccgtgatcatcaccagcaccagcagctactacgtgttctacatctacgtgggcgtggccgacaccctgctggccatgggcttcttcagaggcctgcccctggtgcacaccctgatcaccgtgagcaagatcctgcaccacaagatgctgcacagcgtgctgcaggcccccatgagcaccctgaacaccctgaaggccggcggcatcctgaacagattcagcaaggacatcgccatcctggacgacctgctgcccctgaccatcttcgacttcatccagctgctgctgatcgtgatcggcgccatcgccgtggtggccgtgctgcagccctacatcttcgtggccaccgtgcccgtgatcgtggccttcatcatgctgagagcctacttcctgcagaccagccagcagctgaagcagctggagagcgagggcaggagccccatcttcacccacctggtgaccagcctgaagggcctgtggaccctgagagccttcggcagacagccctacttcgagaccctgttccacaaggccctgaacctgcacaccgccaactggttcctgtacctgagcaccctgagatggttccagatgagaatcgagatgatcttcgtgatcttcttcatcgccgtgaccttcatcagcatcctgaccaccggcgagggcgagggcagagtgggcatcatcctgaccctggccatgaacatcatgagcaccctgcagtgggccgtgaacagcagcatcgacgtggacagcctgatgagaagcgtgagcagagtgttcaagttcatcgacatgcccaccgagggcaagcccaccaagagcaccaagccctacaagaacggccagctgagcaaggtgatgatcatcgagaacagccacgtgaagaaggacgacatctggcccagcggcggccagatgaccgtgaaggacctgaccgccaagtacaccgagggcggcaacgccatcctggagaacatcagcttcagcatcagccccggccagagagtgggcctgctgggcagaaccggcagcggcaagagcaccctgctgagcgccttcctgagactgctgaacaccgagggcgagatccagatcgacggcgtgagctgggacagcatcaccctgcagcagtggagaaaggccttcggcgtgatcccccagaaggtgttcatcttcagcggcaccttcagaaagaacctggacccctacgagcagtggagcgaccaggagatctggaaggtggccgacgaggtgggcctgagaagcgtgatcgagcagttccccggcaagctggacttcgtgctggtggacggcggctgcgtgctgagccacggccacaagcagctgatgtgcctggccagaagcgtgctgagcaaggccaagatcctgctgctggacgagcccagcgcccacctggaccccgtgacctaccagatcatcagaagaaccctgaagcaggccttcgccgactgcaccgtgatcctgtgcgagcacagaatcgaggccatgctggagtgccagcagttcctggtgatcgaggagaacaaggtgagacagtacgacagcatccagaagctgctgaacgagagaagcctgttcagacaggccatcagccccagcgacagagtgaagctgttcccccacagaaacagcagcaagtgcaagagcaagccccagatcgccgccctgaaggaggagaccgaggaggaggtgcaggacaccagactgtga

SEQ ID NO: 25 - DNA, 4443 bp, Artificial Sequence
  Chemically synthesized oligonucleotide
atgcagaggtcacctctggaaaaggctagcgtggtcagcaagctatttttttcctggacccgcccgatactcaggaagggctaccgacagcggctggagctgagtgacatttatcagattccctccgtcgattccgctgacaacctgtctgagaaactggagcgggaatgggatagggaactggcgtccaaaaaaaaccccaaactcatcaatgcactccgcagatgcttcttctggcggtttatgttttatggcatattcctgtatctgggggaggtgacgaaagccgtgcagccgctgctgcttggtcgcattatcgcgtcatacgatccagataacaaggaggaaagaagtatcgctatctatctcgggatagggctgtgcctgctcttcattgtgcggactcttctcttgcaccccgccattttcggtctgcatcatataggtatgcagatgagaattgcgatgttctcattgatttacaaaaaaacgcttaagctaagttcaagggtgctagataagatatcgatcggccagctggtgtctctgcttagcaacaacctcaataaattcgacgaaggccttgcactggcccacttcgtgtggatcgcccctctgcaggtggctctgctgatggggttaatatgggagctgttgcaggcctccgctttttgtggcctggggtttctcatcgtgttggccttgtttcaggcagggctgggacgtatgatgatgaaatatagggatcagagggctggcaaaatctctgagcgcctggttattacgagtgaaatgattgagaacatccagtcagtgaaggcctattgctgggaggaggccatggaaaaaatgattgagaacctacgccagactgagctgaagttaaccagaaaagccgcctatgtgcgctactttaacagtagcgcatttttcttctccggttttttcgtggtgtttcttagtgtgttgccgtatgccttaatcaagggaataatactccggaagattttcactaccatcagcttctgtatcgtgttgcggatggccgtcacccggcagtttccctgggcagtacagacttggtacgattctctcggagcaattaacaaaatccaagactttctacaaaagcaggagtacaagaccctggagtacaatctgaccaccacagaagtcgtaatggagaatgtaactgccttctgggaagagggctttggcgaactctttgaaaaggccaagcagaacaataacaaccggaagacctccaacggggacgacagcttatttttcagcaatttttctttgctcgggacccctgtactgaaagatattaactttaagatcgagcgcggacaactcctggctgtcgccggcagcactggagctggaaaaacatcactgcttatggtgataatgggagaactcgaaccaagcgagggaaaaataaagcactctggacggattagtttttgctcccagttctcgtggataatgcctggcaccattaaggagaatatcatctttggagtgagttacgacgaataccggtaccggtccgttatcaaggcttgtcaactcgaggaggacatttctaaattcgccgaaaaagataatatagtgctgggcgaaggaggcattacactgagcgggggtcagagagctcgaattagcctcgcccgagcagtctataaagacgccgatctttacctgctggattccccttttgggtatttggatgttctgacagagaaggaaatctttgaatcatgtgtctgtaaactgatggccaataagactaggattctagtgacttcgaaaatggagcacctgaaaaaagcggacaaaattctgatactccatgaagggtcttcctacttctacggcaccttctcagagttgcagaacttacaacctgatttttcatctaagcttatggggtgcgactcgtttgaccagttctccgctgaaagacgaaacagcatcttaacggaaactcttcacaggttctcattagagggagatgcgccggtgtcctggacagagacaaaaaaacagtctttcaaacagacaggagagtttggcgagaagagaaaaaactcaatcctcaatcccatcaattctattagaaagtttagcatcgtccaaaaaacaccattgcagatgaatgggattgaggaggacagtgatgagcctttggaacgaagactgtccctggtacccgatagcgaacagggtgaggccatccttcctaggatctcggtcataagtacagggcccacactgcaggccaggcgacgtcaaagtgtcctcaatcttatgacgcacagtgtgaatcaggggcagaacatccatcgtaagacgacagcttcaactcgaaaggtcagtctagctccacaagccaatcttacagagctggacatttattcccgccgcctcagtcaggagaccggattggaaatatcagaggaaattaatgaagaggatctgaaggaatgcttctttgatgacatggaatcgatccccgctgttactacctggaacacatatctgagatatattaccgtccataagagcttaatctttgtactgatatggtgcttggtgattttcctggcagaggttgcggcgagtttggtcgtgctatggctccttggaaacactcccctgcaggataaggggaactccactcatagcaggaataacagctatgccgtgatcatcacctctacctcctcttattacgtgttttacatatacgtcggtgttgcggataccctgttggcaatggggttctttagaggactacccctagttcacaccctgatcaccgtttcgaagatcttgcaccacaagatgcttcatagcgttctccaagctcctatgagcacccttaatacactgaaagcaggaggtatccttaaccgcttttccaaagacatcgctatactcgacgatttgctcccattgaccatcttcgacttcattcagctgctcctcattgtgatcggcgccattgccgtggtcgcagtgttacagccatatattttcgtagccaccgtgcccgtcatcgtggcatttatcatgctgcgcgcatatttcttacagacatctcagcaactgaagcagctggaatctgagggcagatctcctatttttacacacctggttaccagcctgaagggcctgtggaccctgcgtgctttcggtcgccaaccctactttgagactctcttccataaggctctgaatttacatactgccaattggttcctataccttagtacccttcggtggttccagatgcggatagaaatgatcttcgtgattttcttcatcgcagtcactttcatctctattttgacgaccggtgagggcgagggcagggtgggcatcattctgactttggccatgaacattatgtcaacactccagtgggccgttaattcaagcattgatgtggattccttgatgcgttccgtcagcagggtatttaaattcatagacatgcccaccgagggcaagccaacaaaatctaccaagccatacaaaaatggccaactaagcaaggtcatgattatcgagaattctcatgtgaaaaaggacgacatttggccttccgggggtcaaatgactgtaaaggacctgacggctaaatacactgagggcggtaatgctatcttggagaacatctctttcagcatctcccctggccagagagtgggactgctcgggcggacaggctccggaaagtctacgctcctttcagcattccttagacttctgaacaccgaaggtgagattcagattgacggggtctcttgggactccatcacacttcagcaatggaggaaggcattcggtgtaatcccccaaaaggtttttatcttctccggaacatttcgtaagaatctggacccgtacgagcagtggtcagatcaggagatctggaaagtagcagacgaggtcgggctacggagcgttattgaacagtttcctggcaaactggacttcgttttggtggacggaggctgtgtgctgagtcacggccataaacaactgatgtgcttagctaggtctgttctcagcaaggcaaagattttactgctggatgaaccaagcgcccaccttgatccagtgacatatcaaatcatcagaagaactcttaaacaggcgttcgccgactgcacagtgatcctgtgtgagcacagaatagaagccatgctggaatgtcaacagtttctcgtgattgaggagaacaaggtgcgccagtacgatagcatccagaagttactcaatgaaaggtcactcttcaggcaggccatctcacccagcgaccgcgttaagctgtttccacaccgaaacagttccaagtgcaaaagtaagccacagattgctgcactgaaggaagagacagaagaagaagttcaggacactcggctctga

SEQ ID NO: 26 - DNA, 4443 bp, Artificial Sequence; identical to SEQ ID NO: 8
  Chemically synthesized oligonucleotide

SEQ ID NO: 27 - DNA, 4443 bp, Artificial Sequence
  Chemically synthesized oligonucelotide
atgcaacggagtcctctggaaaaagcctctgtcgtatctaagcttttcttcagttggacacgcccgattttgagaaagggttatcggcaacgcttggaacttagtgacatctaccaaattccaagtgtagactcagccgataacttgagcgaaaagctcgaacgagagtgggatcgagaactggctagcaaaaaaaatcccaaactcataaatgccctgcgacgctgtttcttttggcgatttatgttttacggtattttcctttatttgggtgaggtcacgaaggctgtacagccactgctgctgggtcgcatcattgcctcttacgaccctgacaacaaagaggagcggtcaatagctatctaccttggtataggactttgcttgctcttcatagtccgcacgttgcttctccaccctgctatatttggtctccatcacattgggatgcaaatgcggatcgcgatgttcagtcttatatataaaaagactcttaaactttccagccgggttctggataagatctctattggtcaactggtatctcttttgtctaacaacctgaataagttcgacgagggccttgcattggcccattttgtatggattgcccctttgcaagtcgccctcctgatgggattgatctgggaactcctgcaagctagtgctttttgcggattgggattcctcatagtccttgcgctctttcaggcgggacttggacgcatgatgatgaagtatcgcgaccaacgagctggcaagatcagtgaacggcttgtaataaccagtgaaatgatagagaacatccagagcgtaaaagcttactgttgggaagaagcgatggaaaagatgattgagaaccttcgccagacagaacttaaacttacacgaaaggccgcttatgtccggtacttcaactcttcagcatttttttttagtggcttctttgtagtgttcctgtccgtccttccgtatgcacttatcaagggtataatacttaggaaaatcttcacaacaatcagtttttgcatagtccttcgcatggcagtaactcgccaatttccctgggcagttcagacgtggtacgactcacttggcgcaattaacaaaattcaagatttcctccaaaagcaagagtataaaaccttggaatacaaccttaccaccacagaagttgtaatggaaaatgtcacagccttctgggaggaaggtttcggcgaactttttgagaaggcgaagcaaaataacaataatcggaaaacatcaaacggtgacgattcactgttcttttctaactttagccttcttgggacgcccgtcctgaaggacataaactttaagattgaacggggtcaacttctcgcggtcgcagggagtactggagcggggaaaacgagcctgctgatggtgataatgggggagttggagccctcagaaggcaagatcaagcatagtggtagaattagcttctgcagtcaatttagttggattatgccgggcacgatcaaagaaaatataatctttggggtatcctacgatgaatacaggtaccgatcagtgataaaagcgtgccagcttgaagaagacatttcaaagtttgctgagaaggataatatcgtacttggagaaggaggtatcaccctgtctgggggtcaacgagcgaggatctccctggcacgcgccgtctacaaggacgcggacctctatctgttggattcaccgttcggatatttggacgtgcttacggagaaagaaatatttgagagctgtgtttgcaagctcatggcaaataaaaccagaatattggttacaagcaagatggagcatcttaagaaagcagataaaatcctgatattgcacgagggctcttcatacttctacgggacgttttctgagttgcagaacctccagccggatttcagctctaagctgatgggctgtgattcctttgatcagtttagtgcggaaagacgaaacagtatactcaccgaaacactgcacaggttctctctggagggcgacgccccggtttcctggacagagacgaagaagcagtccttcaaacagacaggcgagtttggggagaaaaggaaaaatagcatactcaacccgattaacagcattcgcaagttcagtatagtacaaaagaccccgttgcagatgaacggtatagaggaagattctgatgagccactggaaagacggctttctctcgttccggacagtgaacagggagaggcaatactgcctcggatcagcgttatctctacaggacctactttgcaagctcggcgccgacagtcagtcttgaatcttatgactcatagtgttaatcaaggccagaatatccatcgcaagaccaccgcaagtacaaggaaagtgagcttggcacctcaagcaaaccttactgaacttgatatctactcacggcgactttcacaggagaccggacttgaaattagtgaagaaattaacgaggaggacctcaaggagtgcttcttcgatgacatggaatcaatccccgcagtcacaacctggaacacttatctgaggtatataacagttcacaagagcctcatttttgtacttatttggtgtttggtaattttcctggcggaggttgctgcttctttggtcgtcctttggctcctcgggaatacaccgctccaagacaaaggcaactctacccatagtaggaacaattcatatgcagtgattataaccagtacatcatcttattacgttttctatatttatgtcggggtagctgacacgctgttggcgatgggcttctttaggggcctccccttggtacacacccttatcacggtgagtaaaatcctgcatcacaaaatgcttcattctgtactccaagcgccgatgagtacgcttaatacgctgaaagcaggagggatactgaatcggttcagcaaggacatcgccattctggatgacctgcttccattgacaatatttgatttcattcagctccttctcatagttattggagccatagcggtggtggctgtgcttcagccttatatattcgttgccacagttcccgttatagtggcatttataatgctcagggcctactttctccagacttcccagcagttgaagcaactcgaatcagaaggaaggtcacctattttcacacatcttgtgacttccttgaagggcttgtggacgctgcgggccttcggaagacaaccatattttgaaactctcttccacaaagctttgaatcttcatactgcgaactggttcctgtatttgagtactttgcgctggttccagatgaggatagaaatgatattcgttatcttctttatcgcggttacgttcataagtatcctcactacgggggagggtgagggtagagtgggcataatactgaccctcgccatgaacattatgtccaccctgcagtgggcggtaaacagcagcatagatgtggattctttgatgcgcagtgtgagcagggtttttaagtttatcgatatgccgacggaaggaaagcccactaaaagcacgaaaccctataaaaatggacagcttagcaaagtaatgataatcgagaatagccatgtgaaaaaggatgacatatggccttccggaggccaaatgactgttaaagatctgaccgctaaatataccgagggcggcaacgcaatactcgaaaacataagcttttccataagccccggccaacgcgtgggtcttctggggaggactggctccggaaaatcaacgttgcttagcgcgtttttgcggctccttaacactgaaggtgagatccaaatagatggcgttagttgggactctataacactgcaacaatggcggaaagctttcggcgtcatacctcagaaggtgttcatctttagcggaacgttcaggaagaacttggatccctacgaacaatggagtgatcaagaaatatggaaagtggcagatgaggtaggcttgcgcagtgtcattgaacaattcccagggaaactcgactttgtactggtggacggcggttgcgtcttgtcacacgggcacaaacagttgatgtgtttggcccgcagtgttttgtctaaggcgaagattctgttgctcgacgaaccgagtgctcatcttgatcccgtcacctaccaaatcatcagaaggacgttgaagcaagctttcgccgactgcactgtaatcctttgtgagcataggatcgaagcaatgctcgagtgccaacagttcttggttatagaggagaataaggttcggcaatacgactcaatacagaaactgcttaatgagcggtcactctttcgacaagctatctctcctagtgacagggtaaagctttttcctcatcggaattccagcaagtgtaagagtaaaccacagatcgccgcccttaaagaggagaccgaagaagaggtgcaggatacgagactttag